European Patent Specification EP 3 532 610 B1, published September 27, 2023. Title: METHOD FOR PRODUCING ALDEHYDE. Applicant: Ajinomoto Co., Inc. The sequence listing filed with the application follows.

SEQUENCE LISTING (85 sequences)

SEQ ID NO: 1 - DNA, 1071 bp, Escherichia coli
atgcaaaaagacgcgctgaataacgtacatattaccgacgaacaggttttaatgactccggaacaactgaaggccgcttttccattgagcctgcaacaagaagcccagattgctgactcgcgtaaaagcatttcagatattatcgccgggcgcgatcctcgtctgctggtagtatgtggtccttgttccattcatgatccggaaactgctctggaatatgctcgtcgatttaaagcccttgccgcagaggtcagcgatagcctctatctggtaatgcgcgtctattttgaaaaaccccgtaccactgtcggctggaaagggttaattaacgatccccatatggatggctcttttgatgtagaagccgggctgcagatcgcgcgtaaattgctgcttgagctggtgaatatgggactgccactggcgacggaagcgttagatccgaatagcccgcaatacctgggcgatctgtttagctggtcagcaattggtgctcgtacaacggaatcgcaaactcaccgtgaaatggcctccgggctttccatgccggttggttttaaaaacggcaccgacggcagtctggcaacagcaattaacgctatgcgcgccgccgcccagccgcaccgttttgttggcattaaccaggcagggcaggttgcgttgctacaaactcaggggaatccggacggccatgtgatcctgcgcggtggtaaagcgccgaactatagccctgcggatgttgcgcaatgtgaaaaagagatggaacaggcgggactgcgcccgtctctgatggtagattgcagccacggtaattccaataaagattatcgccgtcagcctgcggtggcagaatccgtggttgctcaaatcaaagatggcaatcgctcaattattggtctgatgatcgaaagtaatatccacgagggcaatcagtcttccgagcaaccgcgcagtgaaatgaaatacggtgtatccgtaaccgatgcctgcattagctgggaaatgaccgatgccttgctgcgtgaaattcatcaggatctgaacgggcagctgacggctcgcgtggcttaa

SEQ ID NO: 2 - protein, 356 aa, Escherichia coli
MQKDALNNVHITDEQVLMTPEQLKAAFPLSLQQEAQIADSRKSISDIIAGRDPRLLVVCGPCSIHDPETALEYARRFKALAAEVSDSLYLVMRVYFEKPRTTVGWKGLINDPHMDGSFDVEAGLQIARKLLLELVNMGLPLATEALDPNSPQYLGDLFSWSAIGARTTESQTHREMASGLSMPVGFKNGTDGSLATAINAMRAAAQPHRFVGINQAGQVALLQTQGNPDGHVILRGGKAPNYSPADVAQCEKEMEQAGLRPSLMVDCSHGNSNKDYRRQPAVAESVVAQIKDGNRSIIGLMIESNIHEGNQSSEQPRSEMKYGVSVTDACISWEMTDALLREIHQDLNGQLTARVA

SEQ ID NO: 3 - DNA, 1089 bp, Escherichia coli
atggagaggattgtcgttactctcggggaacgtagttacccaattaccatcgcatctggtttgtttaatgaaccagcttcattcttaccgctgaaatcgggcgagcaggtcatgttggtcaccaacgaaaccctggctcctctgtatctcgataaggtccgcggcgtacttgaacaggcgggtgttaacgtcgatagcgttatcctccctgacggcgagcagtataaaagcctggctgtactcgataccgtctttacggcgttgttacaaaaaccgcatggtcgcgatactacgctggtggcgcttggcggcggcgtagtgggcgatctgaccggcttcgcggcggcgagttatcagcgcggtgtccgtttcattcaagtcccgacgacgttactgtcgcaggtcgattcctccgttggcggcaaaactgcggtcaaccatcccctcggtaaaaacatgattggcgcgttctaccaacctgcttcagtggtggtggatctcgactgtctgaaaacgcttcccccgcgtgagttagcgtcggggctggcagaagtcatcaaatacggcattattcttgacggtgcgttttttaactggctggaagagaatctggatgcgttgttgcgtctggacggtccggcaatggcgtactgtattcgccgttgttgtgaactgaaggcagaagttgtcgccgccgacgagcgcgaaaccgggttacgtgctttactgaatctgggacacacctttggtcatgccattgaagctgaaatggggtatggcaattggttacatggtgaagcggtcgctgcgggtatggtgatggcggcgcggacgtcggaacgtctcgggcagtttagttctgccgaaacgcagcgtattataaccctgctcaagcgggctgggttaccggtcaatgggccgcgcgaaatgtccgcgcaggcgtatttaccgcatatgctgcgtgacaagaaagtccttgcgggagagatgcgcttaattcttccgttggcaattggtaagagtgaagttcgcagcggcgtttcgcacgagcttgttcttaacgccattgccgattgtcaatcagcgtaa

SEQ ID NO: 4 - protein, 362 aa, Escherichia coli
MERIVVTLGERSYPITIASGLFNEPASFLPLKSGEQVMLVTNETLAPLYLDKVRGVLEQAGVNVDSVILPDGEQYKSLAVLDTVFTALLQKPHGRDTTLVALGGGVVGDLTGFAAASYQRGVRFIQVPTTLLSQVDSSVGGKTAVNHPLGKNMIGAFYQPASVVVDLDCLKTLPPRELASGLAEVIKYGIILDGAFFNWLEENLDALLRLDGPAMAYCIRRCCELKAEVVAADERETGLRALLNLGHTFGHAIEAEMGYGNWLHGEAVAAGMVMAARTSERLGQFSSAETQRIITLLKRAGLPVNGPREMSAQAYLPHMLRDKKVLAGEMRLILPLAIGKSEVRSGVSHELVLNAIADCQSA

SEQ ID NO: 5 - DNA, 759 bp, Escherichia coli
atgaaaaccgtaactgtaaaagatctcgtcattggtacgggcgcacctaaaatcatcgtctcgctgatggcgaaagatatcgccagcgtgaaatccgaagctctcgcctatcgtgaagcggactttgatattctggaatggcgtgtggaccactatgccgacctctccaatgtggagtctgtcatggcggcagcaaaaattctccgtgagaccatgccagaaaaaccgctgctgtttaccttccgcagtgccaaagaaggcggcgagcaggcgatttccaccgaggcttatattgcactcaatcgtgcagccatcgacagcggcctggttgatatgatcgatctggagttatttaccggtgatgatcaggttaaagaaaccgtcgcctacgcccacgcgcatgatgtgaaagtagtcatgtccaaccatgacttccataaaacgccggaagccgaagaaatcattgcccgtctgcgcaaaatgcaatccttcgacgccgatattcctaagattgcgctgatgccgcaaagtaccagcgatgtgctgacgttgcttgccgcgaccctggagatgcaggagcagtatgccgatcgtccaattatcacgatgtcgatggcaaaaactggcgtaatttctcgtctggctggtgaagtatttggctcggcggcaacttttggtgcggtaaaaaaagcgtctgcgccagggcaaatctcggtaaatgatttgcgcacggtattaactattttacaccaggcataa

SEQ ID NO: 6 - protein, 252 aa, Escherichia coli
MKTVTVKDLVIGTGAPKIIVSLMAKDIASVKSEALAYREADFDILEWRVDHYADLSNVESVMAAAKILRETMPEKPLLFTFRSAKEGGEQAISTEAYIALNRAAIDSGLVDMIDLELFTGDDQVKETVAYAHAHDVKVVMSNHDFHKTPEAEEIIARLRKMQSFDADIPKIALMPQSTSDVLTLLAATLEMQEQYADRPIITMSMAKTGVISRLAGEVFGSAATFGAVKKASAPGQISVNDLRTVLTILHQA

SEQ ID NO: 7 - DNA, 843 bp, Bacillus thuringiensis
atgaaatattcgctatgtaccatttcatttcgtcatcaattaatttcatttactgatattgttcaatttgcatatgaaaacggttttgaaggaattgaattatgggggacgcatgcacaaaatttgtacatgcaagaacgtgaaacgacagaacgagaattgaattttctaaaggataaaaacttagaaattacgatgataagtgattacttagatatatcattatcagcagattttgaaaaaacgatagagaaaagtgaacaacttgtagtactagctaattggtttaatacgaataaaattcgcacgtttgctgggcaaaaagggagcaaggacttctcggaacaagagagaaaagagtatgtgaagcgaatacgtaagatttgtgatgtgtttgctcagaacaatatgtatgtgctgttagaaacacatcccaatacactaacggacacattgccttctactatagagttattagaagaagtaaaccatccgaatttaaaaataaatcttgattttcttcatatatgggagtctggcgcagatccaatagacagtttccatcgattaaagccgtggacactacattaccattttaagaatatatcttcagcggattatttgcatgtgtttgaacctaataatgtatatgctgcagcaggaagtcgtataggtatggttccgttatttgaaggtattgtaaattatgatgagattattcaggaagtgagaaatacggatctttttgcttccttagaatggtttggacataattcaaaagagatattaaaagaagaaatgaaagtattaataaatagaaaattagaagtagtaacttcgtaa

SEQ ID NO: 8 - protein, 280 aa, Bacillus thuringiensis
MKYSLCTISFRHQLISFTDIVQFAYENGFEGIELWGTHAQNLYMQERETTERELNFLKDKNLEITMISDYLDISLSADFEKTIEKSEQLVVLANWFNTNKIRTFAGQKGSKDFSEQERKEYVKRIRKICDVFAQNNMYVLLETHPNTLTDTLPSTIELLEEVNHPNLKINLDFLHIWESGADPIDSFHRLKPWTLHYHFKNISSADYLHVFEPNNVYAAAGSRIGMVPLFEGIVNYDEIIQEVRNTDLFASLEWFGHNSKEILKEEMKVLINRKLEVVTS

SEQ ID NO: 9 - DNA, 1542 bp, Escherichia coli
atgcgtctggaagtcttttgtgaagaccgactcggtctgacccgcgaattactcgatctactcgtgctaagaggcattgatttacgcggtattgagattgatcccattgggcgaatctacctcaattttgctgaactggagtttgagagtttcagcagtctgatggccgaaatacgccgtattgcgggtgttaccgatgtgcgtactgtcccgtggatgccttccgaacgtgagcatctggcgttgagcgcgttactggaggcgttgcctgaacctgtgctctctgtcgatatgaaaagcaaagtggatatggcgaacccggcgagctgtcagctttttgggcaaaaattggatcgcctgcgcaaccataccgccgcacaattgattaacggctttaattttttacgttggctggaaagcgaaccgcaagattcgcataacgagcatgtcgttattaatgggcagaatttcctgatggagattacgcctgtttatcttcaggatgaaaatgatcaacacgtcctgaccggtgcggtggtgatgttgcgatcaacgattcgtatgggccgccagttgcaaaatgtcgccgcccaggacgtcagcgccttcagtcaaattgtcgccgtcagcccgaaaatgaagcatgttgtcgaacaggcgcagaaactggcgatgctaagcgcgccgctgctgattacgggtgacacaggtacaggtaaagatctctttgcctacgcctgccatcaggcaagccccagagcgggcaaaccttacctggcgctgaactgtgcgtctataccggaagatgcggtcgagagtgaactgtttggtcatgctccggaagggaagaaaggattctttgagcaggcgaacggtggttcggtgctgttggatgaaataggggaaatgtcaccacggatgcaggcgaaattactgcgtttccttaatgatggcactttccgtcgggttggcgaagaccatgaggtgcatgtcgatgtgcgggtgatttgcgctacgcagaagaatctggtcgaactggtgcaaaaaggcatgttccgtgaagatctctattatcgtctgaacgtgttgacgctcaatctgccgccgctacgtgactgtccgcaggacatcatgccgttaactgagctgttcgtcgcccgctttgccgacgagcagggcgtgccgcgtccgaaactggccgctgacctgaatactgtacttacgcgttatgcgtggccgggaaatgtgcggcagttaaagaacgctatctatcgcgcactgacacaactggacggttatgagctgcgtccacaggatattttgttgccggattatgacgccgcaacggtagccgtgggcgaagatgcgatggaaggttcgctggacgaaatcaccagccgttttgaacgctcggtattaacccagctttatcgcaattatcccagcacgcgcaaactggcaaaacgtctcggcgtttcacataccgcgattgccaataagttgcgggaatatggtctgagtcagaagaagaacgaagagtaa

SEQ ID NO: 10 - protein, 513 aa, Escherichia coli
MRLEVFCEDRLGLTRELLDLLVLRGIDLRGIEIDPIGRIYLNFAELEFESFSSLMAEIRRIAGVTDVRTVPWMPSEREHLALSALLEALPEPVLSVDMKSKVDMANPASCQLFGQKLDRLRNHTAAQLINGFNFLRWLESEPQDSHNEHVVINGQNFLMEITPVYLQDENDQHVLTGAVVMLRSTIRMGRQLQNVAAQDVSAFSQIVAVSPKMKHVVEQAQKLAMLSAPLLITGDTGTGKDLFAYACHQASPRAGKPYLALNCASIPEDAVESELFGHAPEGKKGFFEQANGGSVLLDEIGEMSPRMQAKLLRFLNDGTFRRVGEDHEVHVDVRVICATQKNLVELVQKGMFREDLYYRLNVLTLNLPPLRDCPQDIMPLTELFVARFADEQGVPRPKLAADLNTVLTRYAWPGNVRQLKNAIYRALTQLDGYELRPQDILLPDYDAATVAVGEDAMEGSLDEITSRFERSVLTQLYRNYPSTRKLAKRLGVSHTAIANKLREYGLSQKKNEE

SEQ ID NO: 11 - DNA, 2304 bp, Homo sapiens
cggcctgcgtccgccaccggaagcgccctcctaatccccgcagcgccaccgccattgccgccatcgtcgtggggcttctggggcagctagggctgcccgccgcgctgcctgcgccggaccggggcgggtccagtcccgggcgggccgtcgcgggagagaaataacatctgctttgctgccgagctcagaggagaccccagacccctcccgcagccagagggctggagcctgctcagaggtgctttgaagatgccggaggccccgcctctgctgttggcagctgtgttgctgggcctggtgctgctggtggtgctgctgctgcttctgaggcactggggctggggcctgtgccttatcggctggaacgagttcatcctgcagcccatccacaacctgctcatgggtgacaccaaggagcagcgcatcctgaaccacgtgctgcagcatgcggagcccgggaacgcacagagcgtgctggaggccattgacacctactgcgagcagaaggagtgggccatgaacgtgggcgacaagaaaggcaagatcgtggacgccgtgattcaggagcaccagccctccgtgctgctggagctgggggcctactgtggctactcagctgtgcgcatggcccgcctgctgtcaccaggggcgaggctcatcaccatcgagatcaaccccgactgtgccgccatcacccagcggatggtggatttcgctggcgtgaaggacaaggtcacccttgtggttggagcgtcccaggacatcatcccccagctgaagaagaagtatgatgtggacacactggacatggtcttcctcgaccactggaaggaccggtacctgccggacacgcttctcttggaggaatgtggcctgctgcggaaggggacagtgctactggctgacaacgtgatctgcccaggtgcgccagacttcctagcacacgtgcgcgggagcagctgctttgagtgcacacactaccaatcgttcctggaatacagggaggtggtggacggcctggagaaggccatctacaagggcccaggcagcgaagcagggccctgactgcccccccggcccccctctcgggctctctcacccagcctggtactgaaggtgccagacgtgctcctgctgaccttctgcggctccgggctgtgtcctaaatgcaaagcacacctcggccgaggcctgcgccctgacatgctaacctctctgaactgcaacactggattgttcttttttaagactcaatcatgacttctttactaacactggctagctatattatcttatatactaatatcatgttttaaaaatataaaatagaaattaagaatctaaatatttagatataactcgacttagtacatccttctcaactgccattcccctgctgcccttgacttgggcaccaaacattcaaagctccccttgacggacgctaacgctaagggcggggcccctagctggctgggttctgggtggcacgcctggcccactggcctcccagccacagtggtgcagaggtcagccctcctgcagctaggccaggggcacctgttagccccatggggacgactgccggcctgggaaacgaagaggagtcagccagcattcacacctttctgaccaagcaggcgctggggacaggtggaccccgcagcagcaccagcccctctgggccccatgtggcacagagtggaagcatctccttccctactccccactgggccttgcttacagaagaggcaatggctcagaccagctcccgcatccctgtagttgcctccctggcccatgagtgaggatgcagtgctggtttctgcccacctacacctagagctgtccccatctcctccaaggggtcagactgctagccacctcagaggctccaagggcccagttcccaggcccaggacaggaatcaaccctgtgctagctgagttcacctgcaccgagaccagcccctagccaagattctactcctgggctcaaggcctggctagcccccagccagcccactcctatggatagacagaccagtgagcccaagtggacaagtttggggccacccagggaccagaaacagagcctctgcaggacacagcagatgggcacctgggaccacctccacccagggccctgccccagacgcgcagaggcccgacacaagggagaagccagccacttgtgccagacctgagtggcagaaagcaaaaagttcctttgctgctttaatttttaaattttcttacaaaaatttaggtgtttaccaatagtcttattttggcttatttttaa

SEQ ID NO: 12 - DNA, 2262 bp, Homo sapiens
ctcccacgggaggagcaagaacacagaacagagggggcaagacagctccaccaggagtcaggagtgaatcccctctgggaacgaggcactaggaagaagaacttccagcccaggagaaataacatctgctttgctgccgagctcagaggagaccccagacccctcccgcagccagagggctggagcctgctcagaggtgctttgaagatgccggaggccccgcctctgctgttggcagctgtgttgctgggcctggtgctgctggtggtgctgctgctgcttctgaggcactggggctggggcctgtgccttatcggctggaacgagttcatcctgcagcccatccacaacctgctcatgggtgacaccaaggagcagcgcatcctgaaccacgtgctgcagcatgcggagcccgggaacgcacagagcgtgctggaggccattgacacctactgcgagcagaaggagtgggccatgaacgtgggcgacaagaaaggcaagatcgtggacgccgtgattcaggagcaccagccctccgtgctgctggagctgggggcctactgtggctactcagctgtgcgcatggcccgcctgctgtcaccaggggcgaggctcatcaccatcgagatcaaccccgactgtgccgccatcacccagcggatggtggatttcgctggcgtgaaggacaaggtcacccttgtggttggagcgtcccaggacatcatcccccagctgaagaagaagtatgatgtggacacactggacatggtcttcctcgaccactggaaggaccggtacctgccggacacgcttctcttggaggaatgtggcctgctgcggaaggggacagtgctactggctgacaacgtgatctgcccaggtgcgccagacttcctagcacacgtgcgcgggagcagctgctttgagtgcacacactaccaatcgttcctggaatacagggaggtggtggacggcctggagaaggccatctacaagggcccaggcagcgaagcagggccctgactgcccccccggcccccctctcgggctctctcacccagcctggtactgaaggtgccagacgtgctcctgctgaccttctgcggctccgggctgtgtcctaaatgcaaagcacacctcggccgaggcctgcgccctgacatgctaacctctctgaactgcaacactggattgttcttttttaagactcaatcatgacttctttactaacactggctagctatattatcttatatactaatatcatgttttaaaaatataaaatagaaattaagaatctaaatatttagatataactcgacttagtacatccttctcaactgccattcccctgctgcccttgacttgggcaccaaacattcaaagctccccttgacggacgctaacgctaagggcggggcccctagctggctgggttctgggtggcacgcctggcccactggcctcccagccacagtggtgcagaggtcagccctcctgcagctaggccaggggcacctgttagccccatggggacgactgccggcctgggaaacgaagaggagtcagccagcattcacacctttctgaccaagcaggcgctggggacaggtggaccccgcagcagcaccagcccctctgggccccatgtggcacagagtggaagcatctccttccctactccccactgggccttgcttacagaagaggcaatggctcagaccagctcccgcatccctgtagttgcctccctggcccatgagtgaggatgcagtgctggtttctgcccacctacacctagagctgtccccatctcctccaaggggtcagactgctagccacctcagaggctccaagggcccagttcccaggcccaggacaggaatcaaccctgtgctagctgagttcacctgcaccgagaccagcccctagccaagattctactcctgggctcaaggcctggctagcccccagccagcccactcctatggatagacagaccagtgagcccaagtggacaagtttggggccacccagggaccagaaacagagcctctgcaggacacagcagatgggcacctgggaccacctccacccagggccctgccccagacgcgcagaggcccgacacaagggagaagccagccacttgtgccagacctgagtggcagaaagcaaaaagttcctttgctgctttaatttttaaattttcttacaaaaatttaggtgtttaccaatagtcttattttggcttatttttaa

SEQ ID NO: 13 - DNA, 2279 bp, Homo sapiens
tggagataacacggatcgctgtgtacactgtgtgctccggttgttgcatccgagggttgatcggatggtggttcccatccagatccaagtcctggcccctgatcacagagaaacacagctggacattaaagtgaaataacatctgctttgctgccgagctcagaggagaccccagacccctcccgcagccagagggctggagcctgctcagaggtgctttgaagatgccggaggccccgcctctgctgttggcagctgtgttgctgggcctggtgctgctggtggtgctgctgctgcttctgaggcactggggctggggcctgtgccttatcggctggaacgagttcatcctgcagcccatccacaacctgctcatgggtgacaccaaggagcagcgcatcctgaaccacgtgctgcagcatgcggagcccgggaacgcacagagcgtgctggaggccattgacacctactgcgagcagaaggagtgggccatgaacgtgggcgacaagaaaggcaagatcgtggacgccgtgattcaggagcaccagccctccgtgctgctggagctgggggcctactgtggctactcagctgtgcgcatggcccgcctgctgtcaccaggggcgaggctcatcaccatcgagatcaaccccgactgtgccgccatcacccagcggatggtggatttcgctggcgtgaaggacaaggtcacccttgtggttggagcgtcccaggacatcatcccccagctgaagaagaagtatgatgtggacacactggacatggtcttcctcgaccactggaaggaccggtacctgccggacacgcttctcttggaggaatgtggcctgctgcggaaggggacagtgctactggctgacaacgtgatctgcccaggtgcgccagacttcctagcacacgtgcgcgggagcagctgctttgagtgcacacactaccaatcgttcctggaatacagggaggtggtggacggcctggagaaggccatctacaagggcccaggcagcgaagcagggccctgactgcccccccggcccccctctcgggctctctcacccagcctggtactgaaggtgccagacgtgctcctgctgaccttctgcggctccgggctgtgtcctaaatgcaaagcacacctcggccgaggcctgcgccctgacatgctaacctctctgaactgcaacactggattgttcttttttaagactcaatcatgacttctttactaacactggctagctatattatcttatatactaatatcatgttttaaaaatataaaatagaaattaagaatctaaatatttagatataactcgacttagtacatccttctcaactgccattcccctgctgcccttgacttgggcaccaaacattcaaagctccccttgacggacgctaacgctaagggcggggcccctagctggctgggttctgggtggcacgcctggcccactggcctcccagccacagtggtgcagaggtcagccctcctgcagctaggccaggggcacctgttagccccatggggacgactgccggcctgggaaacgaagaggagtcagccagcattcacacctttctgaccaagcaggcgctggggacaggtggaccccgcagcagcaccagcccctctgggccccatgtggcacagagtggaagcatctccttccctactccccactgggccttgcttacagaagaggcaatggctcagaccagctcccgcatccctgtagttgcctccctggcccatgagtgaggatgcagtgctggtttctgcccacctacacctagagctgtccccatctcctccaaggggtcagactgctagccacctcagaggctccaagggcccagttcccaggcccaggacaggaatcaaccctgtgctagctgagttcacctgcaccgagaccagcccctagccaagattctactcctgggctcaaggcctggctagcccccagccagcccactcctatggatagacagaccagtgagcccaagtggacaagtttggggccacccagggaccagaaacagagcctctgcaggacacagcagatgggcacctgggaccacctccacccagggccctgccccagacgcgcagaggcccgacacaagggagaagccagccacttgtgccagacctgagtggcagaaagcaaaaagttcctttgctgctttaatttttaaattttcttacaaaaatttaggtgtttaccaatagtcttattttggcttatttttaa

SEQ ID NO: 14 - DNA, 2035 bp, Homo sapiens
gctgttggcagctgtgttgctgggcctggtgctgctggtggtgctgctgctgcttctgaggcactggggctggggcctgtgccttatcggctggaacgagttcatcctgcagcccatccacaacctgctcatgggtgacaccaaggagcagcgcatcctgaaccacgtgctgcagcatgcggagcccgggaacgcacagagcgtgctggaggccattgacacctactgcgagcagaaggagtgggccatgaacgtgggcgacaagaaaggcaagatcgtggacgccgtgattcaggagcaccagccctccgtgctgctggagctgggggcctactgtggctactcagctgtgcgcatggcccgcctgctgtcaccaggggcgaggctcatcaccatcgagatcaaccccgactgtgccgccatcacccagcggatggtggatttcgctggcgtgaaggacaaggtcacccttgtggttggagcgtcccaggacatcatcccccagctgaagaagaagtatgatgtggacacactggacatggtcttcctcgaccactggaaggaccggtacctgccggacacgcttctcttggaggaatgtggcctgctgcggaaggggacagtgctactggctgacaacgtgatctgcccaggtgcgccagacttcctagcacacgtgcgcgggagcagctgctttgagtgcacacactaccaatcgttcctggaatacagggaggtggtggacggcctggagaaggccatctacaagggcccaggcagcgaagcagggccctgactgcccccccggcccccctctcgggctctctcacccagcctggtactgaaggtgccagacgtgctcctgctgaccttctgcggctccgggctgtgtcctaaatgcaaagcacacctcggccgaggcctgcgccctgacatgctaacctctctgaactgcaacactggattgttcttttttaagactcaatcatgacttctttactaacactggctagctatattatcttatatactaatatcatgttttaaaaatataaaatagaaattaagaatctaaatatttagatataactcgacttagtacatccttctcaactgccattcccctgctgcccttgacttgggcaccaaacattcaaagctccccttgacggacgctaacgctaagggcggggcccctagctggctgggttctgggtggcacgcctggcccactggcctcccagccacagtggtgcagaggtcagccctcctgcagctaggccaggggcacctgttagccccatggggacgactgccggcctgggaaacgaagaggagtcagccagcattcacacctttctgaccaagcaggcgctggggacaggtggaccccgcagcagcaccagcccctctgggccccatgtggcacagagtggaagcatctccttccctactccccactgggccttgcttacagaagaggcaatggctcagaccagctcccgcatccctgtagttgcctccctggcccatgagtgaggatgcagtgctggtttctgcccacctacacctagagctgtccccatctcctccaaggggtcagactgctagccacctcagaggctccaagggcccagttcccaggcccaggacaggaatcaaccctgtgctagctgagttcacctgcaccgagaccagcccctagccaagattctactcctgggctcaaggcctggctagcccccagccagcccactcctatggatagacagaccagtgagcccaagtggacaagtttggggccacccagggaccagaaacagagcctctgcaggacacagcagatgggcacctgggaccacctccacccagggccctgccccagacgcgcagaggcccgacacaagggagaagccagccacttgtgccagacctgagtggcagaaagcaaaaagttcctttgctgctttaatttttaaattttcttacaaaaatttaggtgtttaccaatagtcttattttggcttatttttaa

SEQ ID NO: 15 - protein, 271 aa, Homo sapiens
MPEAPPLLLAAVLLGLVLLVVLLLLLRHWGWGLCLIGWNEFILQPIHNLLMGDTKEQRILNHVLQHAEPGNAQSVLEAIDTYCEQKEWAMNVGDKKGKIVDAVIQEHQPSVLLELGAYCGYSAVRMARLLSPGARLITIEINPDCAAITQRMVDFAGVKDKVTLVVGASQDIIPQLKKKYDVDTLDMVFLDHWKDRYLPDTLLLEECGLLRKGTVLLADNVICPGAPDFLAHVRGSSCFECTHYQSFLEYREVVDGLEKAIYKGPGSEAGP

SEQ ID NO: 16 - protein, 221 aa, Homo sapiens
MGDTKEQRILNHVLQHAEPGNAQSVLEAIDTYCEQKEWAMNVGDKKGKIVDAVIQEHQPSVLLELGAYCGYSAVRMARLLSPGARLITIEINPDCAAITQRMVDFAGVKDKVTLVVGASQDIIPQLKKKYDVDTLDMVFLDHWKDRYLPDTLLLEECGLLRKGTVLLADNVICPGAPDFLAHVRGSSCFECTHYQSFLEYREVVDGLEKAIYKGPGSEAGP

SEQ ID NO: 17 - DNA, 3387 bp, Gordonia effusa
atgtctgaccagcccaacgcgcttccgtctgccatcgagccgctgaaccccgatcctcaagcgacagagcagatctcgcactgtgcgacgattgccgaacttgtccgggttctcgccgagagctacggtgatcgccccgcgctgggttggcgaaacaatagtgatccctcgtcctggcattcgatgacttaccgagatctcgctgagcgggcggattccatggcgcgacttctccattcgacacttggcgtcgccgagaacgaccgggtggcgacggtgggcttcactagcgcggagtacaccatcgcctcgcttgccgtcggcacgctcggcgcgatggaggtaccactgcaaaacgccgggtccgtcgacgtctgggccgcaatcctcaccgaaaccgactgtgtgagcgcggttgtcgcggccgatcaactgccttcgatcgctcggctggccgaatcgggcacctacaccggcctgcgacatgtgctggtcttcgacatcggctcgcgcgacggaaccacgctcgatgacgcggcacgacgactggtcgctgcgggcacccaggtgcatctccgccagcccggcgccgagccgacgacaccgccggctccactgccccagatcacggccaaccccgaccgcgtcgccctcctcatctacacctccggtagcaccggagcccccaaaggcgccatgtacaccgaaaccgcggtgacccggttattccaatcgggactcagcggcttggggcgcgccaccgacggtcacggctggatcaccctgaacttcatgccgatgagccacgtgatgggacgcagcactctgtggcaaaccctgggaaatggtggcaccgcgtacttcaccccgcgcgccgacctcgccgagttgctcaccgacctcgcagcggtccagccgaccgacctgcaattcgtaccgcgcatctgggacatgctgtaccaggagtacgtccgcctcaccgatcaggacgtcagtgaacaagacgccctcacccgtatgcgcgaacactatttcggtacccggactgccaccgccatcaccggttccgcaccgatctccgatgaggttcggcgtttcgtcgaagcgatgctgccggttccactcatcgaaggctatggaagtaccgaggccgccggcgtctccatcgacggccgcatccagcgaccgccggtggtggattacaagcttctcgacgttcctgaactcggctacctgagcaccgatcggccgcacccgcgcggcgaactgctcgtcaagaccgaccatatcttcgcggggtactacaaccgtcccgacctcacctcatcggtcttcgacgaccagggctactaccggacgggcgacatcgtcgccgagaccggcccagaccaaatcgagtatgtcgaccgccggaacaacgtgatgaagctttcgcagggtgagttcgtcgcgatcgcccacatcgaggcggtactgaccaccccgccgatccagcaactgtacgtctacggcaacagcgcgcggccctatctgctcgcggtcgtcgtgcccacccccgagttacgcgaacgacacgccgacgacaacgagctgcgacgagaagtactgacggcactgcgctctcatggcgaacgtaatggccttgcggccgtagagattccgcgcgatgtgattgtcgaacgcacgccgttcagcctggagaacggtcttcttaccggcatccgaaaactcgcgcgcccacaactcaaagagcgctacggcgctcggctggaggccctctacgccgagctggccgatagccgtatcaccaggctgcgcgacgtcaaagccgttgccgcacaacgctcaacggtgacaacggtcatcgacgtggtcacagcgatactcgacctcgccgacggggaggtcacggccgcggcacatttcaccgacctcggcggagattccctcaccgccgtcacggtcgggaacgaactccgcgacatcttcgacgccgaagtaccggtcggcgtcttgaccagcccgtcatcgacgctggccgacatagccgaacatatcgacgggcgacacagcgaggcccggccaaccgcggaatcggtccacggcaccggaaccacccttcgggcagcggacctcactctcgacaaattcctcgacgaggagaccttgcgcgctgcgtccgacgtgacgtcggctgcgaccgacgtacggaccgtattcatcaccggcgcaaccggattcctcggtcgctatctgacactcgactggttgcgtcggatggcaaaagtcggcggcacggtgatctgcctcgttcgaggtgcggacgatgatgccgcccgggcgcgcctagacgcggcattcgactccagcgatctatggtcggagtaccagcgactggccaaagaccaccttcgggttctcgccggcgacaaggactcggatcacctcgcgctcaccccagacgtatgggatgaattggcaaagtccgtcgacctcatcatcgatcccgcggcgctggtcaaccatgtgttgccatatcgagaactattcggacccaacgtatctggcactgctgagctgatcagactcgcggtgacgaccacccgtaagccatacgtgtatatctcaacggtcggtgtaggcgaccaggtcgcgccgggatctttcaccgaggaccccgacatccgcgagatgagctcggtacgcgagattaacgacacttacgccaacggatatggcaacagcaaatgggccggcgaagtattgctcgcgcaggcgcacgaacgatttgagttaccggtcagcgtctttcgctgcgacatgatcgtcgccgatgatcacaccatcgggcagctgaacctacctgacatgttcacgcggctactgatgagcgtgctcgccaccggcttggcacctcgctctttctatcaactcgccaccgacggatcggcacaggaggcccacttcgatgctctgccggtcgatttcctcgccgaagcgatcaacaccctgtgggttaaggacggagcccgcaccttcaacgcgatgaacccgcacgccgacggcatcggattcgatcagtacattcgctggctgatcgacagcggcgagcagatcagccttgtagacaactatgacgattggtatcggcgattcggtgcggccctcgccgatctgccggaaaagcagcgacgcggatcgttgattccgttgctgcacaactatgttcacccgatgacgccgcacaatcgcggtatggcgtcggcggaccgattccacgacgcggtccgaaccgctggcgtcgggcagtcgtccgacatcccgcatatcacgccacagatcatcgagaactacgcccgcagcctccgcggtctcggggtgatctga

SEQ ID NO: 18 - protein, 1128 aa, Gordonia effusa
MSDQPNALPSAIEPLNPDPQATEQISHCATIAELVRVLAESYGDRPALGWRNNSDPSSWHSMTYRDLAERADSMARLLHSTLGVAENDRVATVGFTSAEYTIASLAVGTLGAMEVPLQNAGSVDVWAAILTETDCVSAVVAADQLPSIARLAESGTYTGLRHVLVFDIGSRDGTTLDDAARRLVAAGTQVHLRQPGAEPTTPPAPLPQITANPDRVALLIYTSGSTGAPKGAMYTETAVTRLFQSGLSGLGRATDGHGWITLNFMPMSHVMGRSTLWQTLGNGGTAYFTPRADLAELLTDLAAVQPTDLQFVPRIWDMLYQEYVRLTDQDVSEQDALTRMREHYFGTRTATAITGSAPISDEVRRFVEAMLPVPLIEGYGSTEAAGVSIDGRIQRPPVVDYKLLDVPELGYLSTDRPHPRGELLVKTDHIFAGYYNRPDLTSSVFDDQGYYRTGDIVAETGPDQIEYVDRRNNVMKLSQGEFVAIAHIEAVLTTPPIQQLYVYGNSARPYLLAVVVPTPELRERHADDNELRREVLTALRSHGERNGLAAVEIPRDVIVERTPFSLENGLLTGIRKLARPQLKERYGARLEALYAELADSRITRLRDVKAVAAQRSTVTTVIDVVTAILDLADGEVTAAAHFTDLGGDSLTAVTVGNELRDIFDAEVPVGVLTSPSSTLADIAEHIDGRHSEARPTAESVHGTGTTLRAADLTLDKFLDEETLRAASDVTSAATDVRTVFITGATGFLGRYLTLDWLRRMAKVGGTVICLVRGADDDAARARLDAAFDSSDLWSEYQRLAKDHLRVLAGDKDSDHLALTPDVWDELAKSVDLIIDPAALVNHVLPYRELFGPNVSGTAELIRLAVTTTRKPYVYISTVGVGDQVAPGSFTEDPDIREMSSVREINDTYANGYGNSKWAGEVLLAQAHERFELPVSVFRCDMIVADDHTIGQLNLPDMFTRLLMSVLATGLAPRSFYQLATDGSAQEAHFDALPVDFLAEAINTLWVKDGARTFNAMNPHADGIGFDQYIRWLIDSGEQISLVDNYDDWYRRFGAALADLPEKQRRGSLIPLLHNYVHPMTPHNRGMASADRFHDAVRTAGVGQSSDIPHITPQIIENYARSLRGLGVI

SEQ ID NO: 19 - DNA, 4636 bp, Artificial Sequence
  Nucleotide sequence of DNA fragment containing CAR gene of Nocardia brasiliensis (codon-optimized) and entD gene of Escherichia coli
ccaagcttgcatgccagatcgtttagatccgaaggaaaacgtcgaaaagcaatttgcttttcgacgccccaccccgcgcgttttagcgtgtcagtagacgcgtagggtaagtggggtagcggcttgttagatatcttgaaatcggctttcaacagcattgatttcgatgtatttagctggccgtttgagacgcgatgtccacagggtagctggtagtttgaaaatcaacgccgttgcccttaggattcagtaactggcacattttgtaatgcgctagatctgtgtgcccagtcttccaggctgcttatcacagtgaaagcaaaaccaattcgtggctgcgaaagtcgtagccaccacgaagtccaggaggacatacaatggcaactgacagcaggagcgaccgtctacgtaggcggatagctcagctatttgcagaagatgaacaggttaaggcagcagttccggatcaggaagttgttgaagcaattcgtgcacctggtctgcgtctggctcagattatggcaaccgtgatggaacgttacgcagatcgtcctgcagttgggcagcgtgcaagcgaaccggttaccgaaagcgggcgtaccacctttcgtctgttaccggagtttgaaaccctgacctatcgtgaactgtgggcacgtgtgcgtgcagttgcagcagcatggcatggggacgcagagaggcccttacgtgcaggagactttgtcgctctgctggggtttgcaggtattgactatggtaccttagacttagcaaatattcacctgggtttagttaccgttccgctgcaaagcggtgcaactgcaccgcaactggcagcaattctggcagaaaccacccctcgtgttctggcagcaactcctgatcacctggacattgcagtagagctactgaccggaggggcaagcccggagcgtctggttgtctttgactatcgtcctgcagatgatgaccatcgtgcagcattagaaagcgcacgtaggcgtctaagcgatgcaggttcggcagttgttgttgaaaccttagatgcagtccgtgcacgcggtagcgagctaccggcagcaccgctgtttgtccctgcagcagatgaagatccgctggctctgttaatttacaccagcggtagcaccgggacccccaaaggtgcaatgtataccgagaggctgaatcgtactacgtggctgagcggtgcaaagggtgttggtttaaccttaggttatatgccgatgtcgcacatagcaggacgtgcatcatttgcaggggttctggcacgcggtggtaccgtttattttaccgcacgcagcgacatgagcaccctgtttgaggacctggcactggttcgtccgaccgaaatgttttttgttccgcgtgtttgtgacatgatttttcaacgttaccaggcagagctgagccggcgtgcacctgcagcagcagcaagcccggagttagaacaggagctgaaaaccgagctgcgtctaagcgcagtcggagatcgtctattaggggcaattgcaggtagcgcaccgctgagcgcagaaatgcgtgaatttatggaaagcctgctggacctggagctgcatgacggttatggtagcaccgaagcagggattggtgtcctgcaagataacattgttcagaggccgccggttattgactataaattagttgatgttccggagctaggttattttcgtacggatcagccgcaccctcgtggggaactactgctaaagaccgagggaatgataccgggttattttcgtcgtcctgaagttaccgcagaaatttttgacgaagatgggttttacaggaccggggatattgttgcagagttagagccggaccgtctgatttaccttgatcgtcgtaataacgttctgaagctggcacagggtgaatttgttaccgttgcacacctggaggcagtttttgcaacctcgccgctgattcgtcagatttacatttacggtaatagcgaacgtagctttctgctggcagttattgttcctaccgcagatgcactggcagatggggttaccgatgcactgaataccgcactgaccgagagcctaaggcagttagcaaaggaggcaggactgcaaagctacgaactgccgcgtgaatttctggttgagaccgagccgtttaccgtagaaaatgggctgttaagcgggattgcaaagctgctacgtcctaaattaaaagaacattacggtgaaaggttagaacagctgtatcgtgacattgaggcaaatcgtaatgatgaactgattgagctgcgtcgtaccgcagcagaactgccggttttagagaccgtaacccgtgctgctaggagcatgttagggctggcagcaagcgaactacgtccggatgcacactttaccgacttaggtggggactcgctgagcgcactgagcttcagcaccctgctgcaggatatgttagaagttgaagttccggttggggttattgttagccctgcaaatagcttagcagacctggcaaagtatattgaggcagagcgtcacagcggagttcgtcgtccgagcctgattagcgttcatgggcctggtaccgaaattagggcagcagacttaaccctggataaatttattgacgaacgtaccttagctgcagcaaaggcagtcccggcagcaccggcacaggcacagaccgtactgttaaccggagcaaatggttacctgggtcgttttctgtgtctggagtggctgcagaggctggatcagaccggggggaccctggtttgtattgttcgtgggaccgatgcagcagcagcacgcaaacgtctggacgcagtttttgacagcggggacccggagctgttagatcattaccgtaaactggcagcagaacatttagaagttttagcaggtgacattggtgatccgaacttaggtctggatgaggcaacttggcagcgtttagcagcaaccgtcgatctgattgttcatcctgcagcattagttaatcacgttctgccgtatagccagctgtttggaccgaacgttgttggtaccgcagaaattattcgtctggcaattaccgaacgtaggaaacctgttacctatctgagcaccgttgcagttgcagctcaggttgacccggcaggttttgacgaagaacgtgacattcgtgaaatgagcgcagttcgtagcattgacgcaggatatgcaaatgggtatggtaatagcaaatgggcaggtgaagttctgctgcgtgaagcacacgatctgtgtggactgccggttgcagtttttcgtagcgatatgattctggcacatagcaagtatgttgggcagttaaatgttcctgacgtttttacccgtttaattctgagcctggcattaaccgggattgctccgtacagcttttacggaaccgatagcgcaggacagcgtaggcgtgcacattacgacgggctgcctgcagactttgttgcagaagcaattaccaccttaggtgcaagggcagaaagcggatttcacacctatgatgtttggaatccgtatgatgatggtattagcctggatgagtttgttgattggttaggtgactttggtgttccgattcagcgtattgacgactatgatgagtggtttcgtaggtttgaaaccgcaattcgtgcactgcctgagaaacagcgtgacgctagcctgctaccgctgctggatgctcatcgtcgtcccctgcgtgcagttcgtgggagcctgctacctgcaaaaaattttcaagcagcagttcagagcgcacgcattggtcctgaccaggatattccgcacctaagcccgcagctaattgacaaatatgttaccgatctgcgtcatttaggtctgttataaaggaggacatacaatggtcgatatgaaaactacgcatacctccctcccctttgccggacatacgctgcattttgttgagttcgatccggcgaatttttgtgagcaggatttactctggctgccgcactacgcacaactgcaacacgctggacgtaaacgtaaaacagagcatttagccggacggatcgctgctgtttatgctttgcgggaatatggctataaatgtgtgcccgcaatcggcgagctacgccaacctgtctggcctgcggaggtatacggcagtattagccactgtgggactacggcattagccgtggtatctcgtcaaccgattggcattgatatagaagaaattttttctgtacaaaccgcaagagaattgacagacaacattattacaccagcggaacacgagcgactcgcagactgcggtttagccttttctctggcgctgacactggcattttccgccaaagagagcgcatttaaggcaagtgagatccaaactgatgcaggttttctggactatcagataattagctggaataaacagcaggtcatcattcatcgtgagaatgagatgtttgctgtgcactggcagataaaagaaaagatagtcataacgctgtgccaacacgattaattgacaacatctggtacgattcgcccgcagccatcactgaccacgggcgaaagtgtaaagcaggtgccttaccatcctgacctgacaaccggatatgcgggatccccgggtaccg

SEQ ID NO: 20 - DNA, 4522 bp, Artificial Sequence
  Nucleotide sequence of DNA fragment containing CAR gene of Gordonia effusa (codon-optimized) and entD gene of Escherichia coli
ccaagcttgcatgccagatcgtttagatccgaaggaaaacgtcgaaaagcaatttgcttttcgacgccccaccccgcgcgttttagcgtgtcagtagacgcgtagggtaagtggggtagcggcttgttagatatcttgaaatcggctttcaacagcattgatttcgatgtatttagctggccgtttgagacgcgatgtccacagggtagctggtagtttgaaaatcaacgccgttgcccttaggattcagtaactggcacattttgtaatgcgctagatctgtgtgcccagtcttccaggctgcttatcacagtgaaagcaaaaccaattcgtggctgcgaaagtcgtagccaccacgaagtccaggaggacatacaatgagcgatcagccgaatgcactgccgagcgcaattgaaccgctgaatccggatccgcaggcaaccgagcagattagccattgtgcaaccattgcagaactggttcgtgttctggcagaaagctatggtgatcgtccggcactgggttggcgtaataatagcgatccgagcagctggcatagcatgacctatcgtgatctggccgaacgtgcagatagcatggcacgtctgctgcatagcaccctgggtgttgcagaaaatgatcgtgttgcaaccgttggttttaccagcgcagaatataccattgcaagcctggcagttggtacactgggtgcaatggaagttccgctgcagaatgcaggtagcgttgatgtttgggcagcaattctgaccgaaaccgattgtgttagcgcagttgttgcagcagatcagctgccgagcattgcccgtctggcggaaagcggcacctataccggtctgcgtcatgttctggtttttgatattggtagccgtgatggcaccaccctggatgatgcagcacgtcgtctggttgccgcaggcacccaggttcatctgcgtcagcctggtgcagaaccgaccacccctccggcaccgctgccgcagattaccgcaaacccggatcgtgtggcactgctgatttataccagcggtagcacaggtgcaccgaaaggtgcaatgtataccgaaacagcagttacccgtctgtttcagagcggtctgagtggtctgggtcgtgcaaccgatggtcatggttggattaccctgaactttatgccgatgagccatgttatgggtcgtagtaccctgtggcagaccctgggtaatggtggcaccgcatattttacaccgcgtgcagatctggctgaactgctgaccgatctggcagccgttcagccgacggatctgcagtttgttccgcgtatttgggatatgctgtatcaagaatatgttcgtctgacagatcaggatgttagcgaacaggatgcactgacccgtatgcgtgaacattatttcggcacccgtaccgcaaccgcaattaccggtagcgcaccgattagtgatgaagttcgtcgttttgttgaagcaatgctgccggttccgctgattgaaggttatggtagcaccgaagcagccggtgttagcattgatggtcgtattcagcgtccgcctgttgttgattataaactgctggatgtgccggaactgggttatctgagcaccgatcgtccgcatccgcgtggtgagctgctggttaaaaccgatcatatttttgccggttattacaatcgtccggatctgaccagcagcgtttttgatgatcagggttattatcgtaccggtgatattgttgccgaaaccggtccggatcagattgaatatgttgatcgtcgtaacaacgtgatgaaactgagccagggtgaatttgttgcaattgcccatattgaagcagttctgaccaccccaccgattcagcagctgtatgtttatggtaatagcgcacgtccgtatctgctggccgttgttgttccgacaccggaactgcgtgaacgtcatgcagatgataatgaactgcgtcgtgaagttctgacagcactgcgtagccatggtgaacgtaatggtctggcagcagttgaaattccgcgtgatgttattgttgaacgtaccccgtttagcctggaaaatggtctgctgacaggtattcgtaaactggcacgtccgcagctgaaagaacgttatggtgcacgtctggaagcactgtatgccgaactggccgatagccgtattacacgtctgcgtgatgtgaaagcagttgcagcccagcgtagcaccgttaccaccgttattgatgttgttaccgcaattctggatctggcggatggtgaagttaccgcagcagcacattttacagatctgggtggtgatagcctgaccgcagttaccgttggtaacgaactgcgcgatatttttgatgccgaagttccggttggtgtgctgaccagcccgagcagtaccctggcagatattgcggaacatattgatggccgtcatagcgaagcacgtccgaccgcagaaagcgttcatggcaccggtacaaccctgcgtgcagccgatctgaccctggataaatttctggatgaagaaacactgcgtgccgcaagtgatgttaccagtgcagccaccgatgttcgtaccgtgtttattaccggtgcaaccggttttctgggtcgctacctgacactggattggctgcgtcgtatggcaaaagttggtggtacagttatttgtctggtgcgtggtgccgatgatgacgcagcccgtgcgcgtctggatgcagcatttgatagcagcgatctgtggtctgaatatcagcgtctggcaaaagatcatctgcgcgtgctggcaggcgataaagatagcgatcatctggcactgacaccggatgtgtgggatgaactggcaaaaagcgttgatctgattattgatccggcagcactggttaatcatgtactgccgtatcgcgaactgtttggtccgaatgttagcggcaccgcagaactgatccgtctggcagttaccaccacccgtaaaccgtatgtgtatatttcaaccgtgggtgttggtgatcaggttgctccgggtagctttaccgaagatcctgatattcgtgaaatgagcagcgtgcgtgaaatcaatgatacctatgcaaatggttacggcaatagcaaatgggcaggcgaagttctgctggcacaggcacatgaacgttttgaactgccggttagcgtttttcgttgtgatatgattgttgcggatgatcataccattggtcagctgaatctgccggatatgtttactcgcctgctgatgagcgttctggcaacaggtctggcaccgcgtagcttttatcagctggcgaccgatggtagtgcacaagaggcacattttgatgcgctgccggtggatttcctggccgaagcaattaatacactgtgggttaaagatggtgcccgtacctttaatgcaatgaatccgcatgccgatggtattggttttgatcagtatattcgttggctgattgatagcggtgaacaaattagcctggtggataattatgatgattggtatcgtcgctttggtgccgcactggcggatctgcctgaaaaacagcgtcgtggtagcctgattccgctgctgcacaattatgttcatccgatgacaccgcataatcgtggtatggcaagcgcagatcgttttcatgatgcagttcgtacagcaggcgttggtcagagcagcgatattccgcatattacccctcagattattgaaaattatgcacgtagcctgcgtggcctgggtgtgatttaaaggaggacatacaatggtcgatatgaaaactacgcatacctccctcccctttgccggacatacgctgcattttgttgagttcgatccggcgaatttttgtgagcaggatttactctggctgccgcactacgcacaactgcaacacgctggacgtaaacgtaaaacagagcatttagccggacggatcgctgctgtttatgctttgcgggaatatggctataaatgtgtgcccgcaatcggcgagctacgccaacctgtctggcctgcggaggtatacggcagtattagccactgtgggactacggcattagccgtggtatctcgtcaaccgattggcattgatatagaagaaattttttctgtacaaaccgcaagagaattgacagacaacattattacaccagcggaacacgagcgactcgcagactgcggtttagccttttctctggcgctgacactggcattttccgccaaagagagcgcatttaaggcaagtgagatccaaactgatgcaggttttctggactatcagataattagctggaataaacagcaggtcatcattcatcgtgagaatgagatgtttgctgtgcactggcagataaaagaaaagatagtcataacgctgtgccaacacgattaattgacaacatctggtacgattcgcccgcagccatcactgaccacgggcgaaagtgtaaagcaggtgccttaccatcctgacctgacaaccggatatgcgggatccccgggtaccg

SEQ ID NO: 21 - DNA, 621 bp, Escherichia coli
atgaaaactacgcatacctccctcccctttgccggacatacgctgcattttgttgagttcgatccggcgaatttttgtgagcaggatttactctggctgccgcactacgcacaactgcaacacgctggacgtaaacgtaaaacagagcatttagccggacggatcgctgctgtttatgctttgcgggaatatggctataaatgtgtgcccgcaatcggcgagctacgccaacctgtctggcctgcggaggtatacggcagtattagccactgtgggactacggcattagccgtggtatctcgtcaaccgattggcattgatatagaagaaattttttctgtacaaaccgcaagagaattgacagacaacattattacaccagcggaacacgagcgactcgcagactgcggtttagccttttctctggcgctgacactggcattttccgccaaagagagcgcatttaaggcaagtgagatccaaactgatgcaggttttctggactatcagataattagctggaataaacagcaggtcatcattcatcgtgagaatgagatgtttgctgtgcactggcagataaaagaaaagatagtcataacgctgtgccaacacgattaa

SEQ ID NO: 22 - protein, 206 aa, Escherichia coli
MKTTHTSLPFAGHTLHFVEFDPANFCEQDLLWLPHYAQLQHAGRKRKTEHLAGRIAAVYALREYGYKCVPAIGELRQPVWPAEVYGSISHCGTTALAVVSRQPIGIDIEEIFSVQTARELTDNIITPAEHERLADCGLAFSLALTLAFSAKESAFKASEIQTDAGFLDYQIISWNKQQVIIHRENEMFAVHWQIKEKIVITLCQHD

SEQ ID NO: 23 - DNA, 654 bp, Corynebacterium glutamicum
atgctggatgagtctttgtttccaaattcggcaaagttttctttcattaaaactggcgatgctgttaatttagaccatttccatcagttgcatccgttggaaaaggcactggtagcgcactcggttgatattagaaaagcagagtttggagatgccaggtggtgtgcacatcaggcactccaagctttgggacgagatagcggtgatcccattttgcgtggggaacgaggaatgccattgtggccttcttcggtgtctggttcattgacccacactgacggattccgagctgctgttgtggcgccacgattgttggtgcgttctatgggattggatgccgaacctgcggagccgttgcccaaggatgttttgggttcaatcgctcgggtgggggagattcctcaacttaagcgcttggaggaacaaggtgtgcactgcgcggatcgcctgctgttttgtgccaaggaagcaacatacaaagcgtggttcccgctgacgcataggtggcttggttttgaacaagctgagatcgacttgcgtgatgatggcacttttgtgtcctatttgctggttcgaccaactccagtgccgtttatttcaggtaaatgggtactgcgtgatggttatgtcatagctgcgactgcagtgacttga

SEQ ID NO: 24 - protein, 217 aa, Corynebacterium glutamicum
MLDESLFPNSAKFSFIKTGDAVNLDHFHQLHPLEKALVAHSVDIRKAEFGDARWCAHQALQALGRDSGDPILRGERGMPLWPSSVSGSLTHTDGFRAAVVAPRLLVRSMGLDAEPAEPLPKDVLGSIARVGEIPQLKRLEEQGVHCADRLLFCAKEATYKAWFPLTHRWLGFEQAEIDLRDDGTFVSYLLVRPTPVPFISGKWVLRDGYVIAATAVT

SEQ ID NO: 25 - DNA, 1428 bp, Corynebacterium glutamicum
atgcgcctgcgtgtctcgagtagtctcctccccttcctcgtccccaacctcgaccattacggtcgccctctcctaaaggagcctggcatggatatccgccaaacaattaacgacacagcaatgtcgagatatcagtggttcattgtatttatcgcagtgctgctcaacgcactggacggctttgatgtcctcgccatgtcttttactgcgaatgcagtgaccgaagaatttggactgagtggcagccagcttggtgtgctgctgagttccgcgctgttcggcatgaccgctggatctttgctgttcggtccgatcggtgaccgtttcggccgtaagaatgccctgatgatcgcgctgctgttcaacgtggtgggattggtattgtccgccaccgcgcagtccgcaggccagttgggcgtgtggcgtttgatcactggtatcggcatcggcggaatcctcgcctgcatcacagtggtgatcagtgagttctccaacaacaaaaaccgcggcatggccatgtccatctacgctgctggttacggcatcggcgcgtccttgggcggattcggcgcagcgcagctcatcccaacatttggatggcgctccgtgttcgcagccggtgcgatcgcaactggtatcgccaccatcgctactttcttcttcctgccagaatccgttgattggctgagcactcgccgccctgcgggcgctcgcgacaagatcaattacattgcgcgccgcctgggcaaagtcggtacctttgagcttccaggcgaacaaagcttgtcgacgaaaaaagccggtctccaatcgtatgcagtgctcgttaacaaagagaaccgtggaaccagcatcaagctgtgggttgcgttcggcatcgtgatgttcggcttctacttcgccaacacttggaccccgaagctgctcgtggaaaccggaatgtcagaacagcagggcatcatcggtggtttgatgttgtccatgggtggagcattcggttccctgctctacggtttcctcaccaccaagttcagctcccgaaacacactgatgaccttcatggtgctgtccggcctgacgctgatcctgttcatttcctccacctctgttccatccatcgcgtttgccagcggcgttgtcgtgggcatgctgatcaatggttgtgtggctggtctgtacaccctgtccccacagctgtactccgctgaagtacgcaccactggtgtgggcgctgcgattggtatgggtcgtgtcggtgcgatttccgcgccactgctggtgggtagcctgctggattctggctggtccccaacgcagctgtatgttggtgtggcagtgattgttattgccggtgcaaccgcattgattgggatgcgcactcaggcagtagccgtcgaaaagcagcctgaagccctagcgaccaaatag

SEQ ID NO: 26 - protein, 475 aa, Corynebacterium glutamicum
MRLRVSSSLLPFLVPNLDHYGRPLLKEPGMDIRQTINDTAMSRYQWFIVFIAVLLNALDGFDVLAMSFTANAVTEEFGLSGSQLGVLLSSALFGMTAGSLLFGPIGDRFGRKNALMIALLFNVVGLVLSATAQSAGQLGVWRLITGIGIGGILACITVVISEFSNNKNRGMAMSIYAAGYGIGASLGGFGAAQLIPTFGWRSVFAAGAIATGIATIATFFFLPESVDWLSTRRPAGARDKINYIARRLGKVGTFELPGEQSLSTKKAGLQSYAVLVNKENRGTSIKLWVAFGIVMFGFYFANTWTPKLLVETGMSEQQGIIGGLMLSMGGAFGSLLYGFLTTKFSSRNTLMTFMVLSGLTLILFISSTSVPSIAFASGVVVGMLINGCVAGLYTLSPQLYSAEVRTTGVGAAIGMGRVGAISAPLLVGSLLDSGWSPTQLYVGVAVIVIAGATALIGMRTQAVAVEKQPEALATK

SEQ ID NO: 27 - DNA, 1296 bp, Corynebacterium glutamicum
gtgtcaacgaccaccccaacccgcgcaaccaaaagtgtcggaacagttctcgcactcctgtggttcgcaattgtcctcgacggctttgacctagtcgtcctgggcgcaacaatcccgtccatgctggaggatcccgcgtgggatctcactgctggacaggccacacagatttccaccatcggcctcgtcggcatgaccatcggcgcactgaccattggtttcttaactgaccgtctgggtcgacgccgcgtcatgctgttctctgtggcagtgttttctgtattcaccctcctgctggcattcaccaccaacgtccagctcttcagcctgtggcgtttcctcgcaggtgttggccttggtggagcactccccaccgcaattgccatggtgaccgagtttcgccccggcaccaaagcgggctctgcatcaactaccttgatgaccggataccacgtcggggcagtagcaaccgctttccttggtctcttccttatcgacggctttggttggcactccatgttcatcgcaggcgctgtgccaggactactcctgctgccactgctgtatttcttccttccagaatccccgcagtacctcaaaatctccggcaagttggatgaggcgcaggcagttgcagcatcttatggactttccctggatgatgatcttgatcgcgaacacgaagaagaacttggcgagtcctcctcactttcctccctgttcaagccctcgttccgccgcaacaccctggcgatttggggcacctcattcatgggactcctcctggtctacggcctgaacacatggctgccacaaatcatgcgccaagcagactacgacatgggtaactccctgggcttcctcatggttcttaacatcggcgcagtgatcggcctttatattgcagggcgaattgccgataagaactcccctcgcaaaacagcactcgtatggttcgtgttctctgcatttttcctcgcactacttgctgtccggatgccactgatcggtctgtatggcatcgtgctgctcaccggcatctttgtgttcagctcccaggtactcatctacgccttcgttggtgagaatcaccctgccaagatgcgtgcaactgccatgggattctccgcaggaattggtcgcctcggcgcgatctcgggtccgttgctgggcggcctgcttgtcagtgccaaccttgcttacccatggggcttcttcgccttcgctggcgttggactgctgggcgcgctgattttctccgcatcgaagactctgaggcatcgcgagaacgcttag

SEQ ID NO: 28 - protein, 431 aa, Corynebacterium glutamicum
MSTTTPTRATKSVGTVLALLWFAIVLDGFDLVVLGATIPSMLEDPAWDLTAGQATQISTIGLVGMTIGALTIGFLTDRLGRRRVMLFSVAVFSVFTLLLAFTTNVQLFSLWRFLAGVGLGGALPTAIAMVTEFRPGTKAGSASTTLMTGYHVGAVATAFLGLFLIDGFGWHSMFIAGAVPGLLLLPLLYFFLPESPQYLKISGKLDEAQAVAASYGLSLDDDLDREHEEELGESSSLSSLFKPSFRRNTLAIWGTSFMGLLLVYGLNTWLPQIMRQADYDMGNSLGFLMVLNIGAVIGLYIAGRIADKNSPRKTALVWFVFSAFFLALLAVRMPLIGLYGIVLLTGIFVFSSQVLIYAFVGENHPAKMRATAMGFSAGIGRLGAISGPLLGGLLVSANLAYPWGFFAFAGVGLLGALIFSASKTLRHRENA

SEQ ID NO: 29 - DNA, 1131 bp, Corynebacterium glutamicum
atgacactgtccgaacgcaagctcaccaccaccgccaagattcttccccacccactcaacgcctggtacgtcgccgcttgggattatgaagtcacatctaaaaagcccatggccaggacaatcgccaacaaaccactcgctttgtaccgcaccaaagatggccgagccgttgcccttgcagacgcctgctggcaccgcctcgcaccgctatccaagggaaaactcgtgggcacagacggaatccaatgcccttatcacggcttggagtacaactccgcgggccgctgcatgaaaatgcccgcgcaggaaaccctcaacccgtcagcagccgtcaactcctaccccgtggtggaagcccaccgctttgtgtgggtgtggctgggcgatcccacattggcagatcccacccaagtacccgatatgcaccagatgagccaccccgaatgggcaggcgatggacgcaccatctccgctgactgcaactaccaattagtgctggacaacttgatggacctcacccacgaagaattcgtgcactcctccagcatcggccaagacgaacttagtgaatcagagttcgtggtcacccacactgaagattccgtgacggtcacccgctggatgcatgacatagatgcaccaccgttttggcaaaagaacatgaatgataagttcccaggatttgaaggcaaggtggatcgttggcagatcatccactactactacccttccaccatctgcattgatgttggtgtagcaaaggctggaaccggcgcgcaggaaggcgaccgcagccagggcgttaatgggtatgtaatgaacaccattaccccagattcagatcgttcctctcattacttctgggcattcatgcgcaactaccgcctggaaagccaaaccatcaccacccagctgcgcgacggtgtatccggtgtattcaaagaagacgaagacatgctgaccgctcagcaagatgccatcgacgccaacaccgactatgagttttacagcctcaacattgatgccggtggcatgtgggtgcgccgaatcctcgaggaagcactctccaaggaaggccgactggatatccccaccacattcccccgcgcaacaccgaagccggaggcataa

SEQ ID NO: 30 - protein, 376 aa, Corynebacterium glutamicum
MTLSERKLTTTAKILPHPLNAWYVAAWDYEVTSKKPMARTIANKPLALYRTKDGRAVALADACWHRLAPLSKGKLVGTDGIQCPYHGLEYNSAGRCMKMPAQETLNPSAAVNSYPVVEAHRFVWVWLGDPTLADPTQVPDMHQMSHPEWAGDGRTISADCNYQLVLDNLMDLTHEEFVHSSSIGQDELSESEFVVTHTEDSVTVTRWMHDIDAPPFWQKNMNDKFPGFEGKVDRWQIIHYYYPSTICIDVGVAKAGTGAQEGDRSQGVNGYVMNTITPDSDRSSHYFWAFMRNYRLESQTITTQLRDGVSGVFKEDEDMLTAQQDAIDANTDYEFYSLNIDAGGMWVRRILEEALSKEGRLDIPTTFPRATPKPEA

SEQ ID NO: 31 - DNA, 978 bp, Corynebacterium glutamicum
atgaactcgcaatggcaagatgcacatgttgtttccagcgaaatcatcgctgcagacattcgacgaatagaactatccccgaaatttgcgattccagtaaaacccggcgaacatctcaagatcatggtgcccctaaaaactggacaggaaaagagatcgtactccatcgttgacgctcgtcacgacggttcgactctcgccctgagcgtactcaaaaccagaaactcccgtggaggatctgagttcatgcatacgcttcgagctggagacacagttactgtctccaggccgtctcaggattttcctctccgcgtgggtgcgcctgagtatgtacttgttgccggcggaattggaatcacagcgatccgttcaatggcatctttattaaagaaattgggagcaaactaccgcattcatttcgcagcacgcagccttgatgccatggcttacaaagatgagctcgtggcagaacacggcgacaagctgcacctgcatctagattctgaaggcaccaccatcgatgtcccagcattgatcgaaaccttaaacccccacactgagctttatatgtgcggccccatccgcttgatggatgccatccggcgcgcatggaacacccgcggacttgaccccaccaatctgcgtttcgaaacgtttggaaacagtggatggttctccccagaggttttccacatccaagtaccagagctggggcttcacgccacagtcaacaaggatgaaagcatgctggaggctttgcaaaaggctggggcgaatatgatgtttgattgtcgaaaaggcgaatgtggtttgtgccaggttcgcgttctagaagtcgatggccaggttgatcaccgcgatgtgttcttctctgatcgtcaaaaagaatccgacgcaaaggcatgcgcctgcgtgtctcgagtagtctcctccccttcctcgtccccaacctcgaccattacggtcgccctctcctaa

SEQ ID NO: 32 - protein, 325 aa, Corynebacterium glutamicum
MNSQWQDAHVVSSEIIAADIRRIELSPKFAIPVKPGEHLKIMVPLKTGQEKRSYSIVDARHDGSTLALSVLKTRNSRGGSEFMHTLRAGDTVTVSRPSQDFPLRVGAPEYVLVAGGIGITAIRSMASLLKKLGANYRIHFAARSLDAMAYKDELVAEHGDKLHLHLDSEGTTIDVPALIETLNPHTELYMCGPIRLMDAIRRAWNTRGLDPTNLRFETFGNSGWFSPEVFHIQVPELGLHATVNKDESMLEALQKAGANMMFDCRKGECGLCQVRVLEVDGQVDHRDVFFSDRQKESDAKACACVSRVVSSPSSSPTSTITVALS

SEQ ID NO: 33 - DNA, 615 bp, Corynebacterium glutamicum
atgattgatacagggaagaacggcgagttccgctacgagcagtcgaatatcatcgatcagaacgaagccgagttcggcatcactccttcacagaccgtgggcccttacgtccacatcggtttgacccttgaaggtgcggagcatctcgtggagccaggttcggaaggcgcggtgtcctttactgtttccgcaactgatggcaacggcgaccccatcgcggatgccatgtttgaactgtggcaggccgatccagagggcatccacaactctgatttggatccaaaccgcacagcaccagcaaccgcagatggcttccgcgggcttggtcgcgcgatggcaaacgcgcagggtgaggcaacgttcaccactttggttccgggagcattcgcagatgaggcaccacacttcaaggttggtgtgttcgcccgtggcatgctggagcgtctgtacactcgcgcatacctgccagacgccgatttgagcaccgacccagttttggctgtggtcccagctgatcgacgtgacctcctggtggctcaaaagaccgatgatggattccgcttcgacatcactgtccaggctgaagacaatgaaaccccattttttggactctaa

SEQ ID NO: 34 - protein, 204 aa, Corynebacterium glutamicum
MIDTGKNGEFRYEQSNIIDQNEAEFGITPSQTVGPYVHIGLTLEGAEHLVEPGSEGAVSFTVSATDGNGDPIADAMFELWQADPEGIHNSDLDPNRTAPATADGFRGLGRAMANAQGEATFTTLVPGAFADEAPHFKVGVFARGMLERLYTRAYLPDADLSTDPVLAVVPADRRDLLVAQKTDDGFRFDITVQAEDNETPFFGL

SEQ ID NO: 35 - DNA, 693 bp, Corynebacterium glutamicum
atggacatcccacacttcgccccgacgggaggcgaatactccccactgcacttcccggagtaccggaccaccatcaagcgcaacccaagcaacgatctcatcatggttcctagtcgcctcggcgagtccacgggacctgtcttcggcgaccgcgacttgggagacatcgacaacgacatgaccaaggtgaacggtggcgaggctatcggccagcgcatcttcgttcacggccgtgtcctcggtttcgatggcaagccagttccgcacaccttggtcgaggcgtggcaggcaaacgccgcaggccgttaccgccacaagaatgactcctggccagcgccactggatccacacttcaacggtgttgcacgtactctcaccgacaaggacggccagtaccacttctggaccgttatgccaggtaattacccttggggtaaccaccacaacgcatggcgcccggcgcacattcacttctcgctctatggtcgtcagtttacggagcgtctggtcacccagatgtacttcccgaacgatccattgttcttccaggatccgatctacaacgcggtgccaaagggtgcacgtgagcgcatgatcgcaacgttcgactatgacgagacccgtgaaaacttcgcgcttggttacaagttcgacatcgtccttcgtggccgcaacgccaccccatttgagtaa

SEQ ID NO: 36 - protein, 230 aa, Corynebacterium glutamicum
MDIPHFAPTGGEYSPLHFPEYRTTIKRNPSNDLIMVPSRLGESTGPVFGDRDLGDIDNDMTKVNGGEAIGQRIFVHGRVLGFDGKPVPHTLVEAWQANAAGRYRHKNDSWPAPLDPHFNGVARTLTDKDGQYHFWTVMPGNYPWGNHHNAWRPAHIHFSLYGRQFTERLVTQMYFPNDPLFFQDPIYNAVPKGARERMIATFDYDETRENFALGYKFDIVLRGRNATPFE

SEQ ID NO: 37 - DNA, 1164 bp, Escherichia coli
atgaacaactttaatctgcacaccccaacccgcattctgtttggtaaaggcgcaatcgctggtttacgcgaacaaattcctcacgatgctcgcgtattgattacctacggcggcggcagcgtgaaaaaaaccggcgttctcgatcaagttctggatgccctgaaaggcatggacgtgctggaatttggcggtattgagccaaacccggcttatgaaacgctgatgaacgccgtgaaactggttcgcgaacagaaagtgactttcctgctggcggttggcggcggttctgtactggacggcaccaaatttatcgccgcagcggctaactatccggaaaatatcgatccgtggcacattctgcaaacgggcggtaaagagattaaaagcgccatcccgatgggctgtgtgctgacgctgccagcaaccggttcagaatccaacgcaggcgcggtgatctcccgtaaaaccacaggcgacaagcaggcgttccattctgcccatgttcagccggtatttgccgtgctcgatccggtttatacctacaccctgccgccgcgtcaggtggctaacggcgtagtggacgcctttgtacacaccgtggaacagtatgttaccaaaccggttgatgccaaaattcaggaccgtttcgcagaaggcattttgctgacgctaatcgaagatggtccgaaagccctgaaagagccagaaaactacgatgtgcgcgccaacgtcatgtgggcggcgactcaggcgctgaacggtttgattggcgctggcgtaccgcaggactgggcaacgcatatgctgggccacgaactgactgcgatgcacggtctggatcacgcgcaaacactggctatcgtcctgcctgcactgtggaatgaaaaacgcgataccaagcgcgctaagctgctgcaatatgctgaacgcgtctggaacatcactgaaggttccgatgatgagcgtattgacgccgcgattgccgcaacccgcaatttctttgagcaattaggcgtgccgacccacctctccgactacggtctggacggcagctccatcccggctttgctgaaaaaactggaagagcacggcatgacccaactgggcgaaaatcatgacattacgttggatgtcagccgccgtatatacgaagccgcccgctaa

SEQ ID NO: 38 - protein, 387 aa, Escherichia coli
MNNFNLHTPTRILFGKGAIAGLREQIPHDARVLITYGGGSVKKTGVLDQVLDALKGMDVLEFGGIEPNPAYETLMNAVKLVREQKVTFLLAVGGGSVLDGTKFIAAAANYPENIDPWHILQTGGKEIKSAIPMGCVLTLPATGSESNAGAVISRKTTGDKQAFHSAHVQPVFAVLDPVYTYTLPPRQVANGVVDAFVHTVEQYVTKPVDAKIQDRFAEGILLTLIEDGPKALKEPENYDVRANVMWAATQALNGLIGAGVPQDWATHMLGHELTAMHGLDHAQTLAIVLPALWNEKRDTKRAKLLQYAERVWNITEGSDDERIDAAIAATRNFFEQLGVPTHLSDYGLDGSSIPALLKKLEEHGMTQLGENHDITLDVSRRIYEAAR

SEQ ID NO: 39 - DNA, 1062 bp, Corynebacterium glutamicum
atgagcatccaagtaaaagcactccagaaaaccggccccgaagcacctttcgaggtcaaaatcattgagcgtcgtgagcctcgcgctgacgacgtagttatcgacatcaaagctgccggcatctgccacagcgatatccacaccatccgcaacgaatggggcgaggcacacttcccgctcaccgtcggccacgaaatcgcaggcgttgtctctgcggttggctccgatgtaaccaagtggaaagtcggcgaccgcgttggcgtcggctgcctagttaactcctgcggcgaatgtgaacagtgtgtcgcgggatttgaaaacaactgccttcgcggaaacgtcggaacctacaactccgacgacgtcgacggcaccatcacgcaaggtggctacgccgaaaaggtagtggtcaacgaacgtttcctctgcagcatcccagaggaactcgacttcgatgtcgcagcaccactgctgtgcgcaggcatcaccacctactccccgatcgctcgctggaacgttaaagaaggcgacaaagtagcagtcatgggcctcggcgggctcggccacatgggtgtccaaatcgccgcagccaagggcgctgacgttaccgttctgtcccgttccctgcgcaaggctgaacttgccaaggaactcggcgcagctcgcacgcttgcgacttctgatgaggatttcttcaccgaacacgccggtgaattcgacttcatcctcaacaccattagcgcatccatcccagtcgacaagtacctgagccttctcaagccacacggtgtcatggctgttgtcggtctgccaccagagaagcagccactgagcttcggtgcgctcatcggcggcggaaaagtcctcaccggatccaacattggcggcatccctgaaacccaggaaatgctcgacttctgtgcaaaacacggcctcggcgcgatgatcgaaactgtcggcgtcaacgatgttgatgcagcctacgaccgcgttgttgccggcgacgttcagttccgcgttgtcattgatactgcttcgtttgcagaggtagaggcggtttag

SEQ ID NO: 40 - protein, 353 aa, Corynebacterium glutamicum
MSIQVKALQKTGPEAPFEVKIIERREPRADDVVIDIKAAGICHSDIHTIRNEWGEAHFPLTVGHEIAGVVSAVGSDVTKWKVGDRVGVGCLVNSCGECEQCVAGFENNCLRGNVGTYNSDDVDGTITQGGYAEKVVVNERFLCSIPEELDFDVAAPLLCAGITTYSPIARWNVKEGDKVAVMGLGGLGHMGVQIAAAKGADVTVLSRSLRKAELAKELGAARTLATSDEDFFTEHAGEFDFILNTISASIPVDKYLSLLKPHGVMAVVGLPPEKQPLSFGALIGGGKVLTGSNIGGIPETQEMLDFCAKHGLGAMIETVGVNDVDAAYDRVVAGDVQFRVVIDTASFAEVEAV

SEQ ID NO: 41 - DNA, 1113 bp, Corynebacterium glutamicum
gtgtccatgagcactgtcgtgcctggaattgtcgccctgtccaagggggcaccggtagaaaaagtaaacgttgttgtccctgatccaggtgctaacgatgtcatcgtcaagattcaggcctgcggtgtgtgccacaccgacttggcctaccgcgatggcgatatttcagatgagttcccttacctcctcggccacgaggcagcaggtattgttgaggaggtaggcgagtccgtcacccacgttgaggtcggcgatttcgtcatcttgaactggcgtgcagtgtgcggcgagtgccgtgcatgtaagaagggcgagccaaagtactgctttaacacccacaacgcatctaagaagatgaccctggaagacggcaccgagctgtccccagcactgggtattggcgcgttcttggaaaagaccctggtccacgaaggccagtgcaccaaggttaaccctgaggaagatccagcagcagctggccttctgggttgcggcatcatggcaggtcttggtgctgcggtaaacaccggtgatattaagcgcggcgagtccgtggcagtcttcggccttggtggcgtgggcatggcagctattgctggcgccaagattgctggtgcatcgaagattattgctgttgatatcgatgagaagaagttggagtgggcgaaggaattcggcgcaacccacaccattaattcctctggtcttggtggcgagggtgatgcctctgaggtcgtggcaaaggttcgtgagctcactgatggtttcggtactgacgtctccatcgatgcggtaggcatcatgccgacctggcagcaggcgttttactcccgtgatcatgcaggccgcatggtgatggtgggcgttccaaacctgacgtctcgcgtagatgttcctgcgattgatttttacggtcgcggtggctctgtgcgccctgcatggtacggcgactgcctgcctgagcgtgatttcccaacttatgtggatctgcacctgcagggtcgtttcccgctggataagtttgtttctgagcgtattggtcttgatgatgttgaagaggctttcaacaccatgaaggctggcgacgtgctgcgttctgtggtggagatctaa

SEQ ID NO: 42 - protein, 370 aa, Corynebacterium glutamicum
MSMSTVVPGIVALSKGAPVEKVNVVVPDPGANDVIVKIQACGVCHTDLAYRDGDISDEFPYLLGHEAAGIVEEVGESVTHVEVGDFVILNWRAVCGECRACKKGEPKYCFNTHNASKKMTLEDGTELSPALGIGAFLEKTLVHEGQCTKVNPEEDPAAAGLLGCGIMAGLGAAVNTGDIKRGESVAVFGLGGVGMAAIAGAKIAGASKIIAVDIDEKKLEWAKEFGATHTINSSGLGGEGDASEVVAKVRELTDGFGTDVSIDAVGIMPTWQQAFYSRDHAGRMVMVGVPNLTSRVDVPAIDFYGRGGSVRPAWYGDCLPERDFPTYVDLHLQGRFPLDKFVSERIGLDDVEEAFNTMKAGDVLRSVVEI

SEQ ID NO: 43 - DNA, 1047 bp, Corynebacterium glutamicum
gtgagttttatgaccactgctgcaccccaagaatttaccgctgctgttgttgaaaaattcggtcatgacgtgaccgtgaaggatattgaccttccaaagccagggccacaccaggcattggtgaaggtactcacctccggcatctgccacaccgacctccacgccttggagggcgattggccagtaaagccggaaccaccattcgtaccaggacacgaaggtgtaggtgaagttgttgagctcggaccaggtgaacacgatgtgaaggtcggcgatattgtcggcaatgcgtggctctggtcagcgtgcggcacctgcgaatactgcatcacaggcagggaaactcagtgtaacgaagctgagtacggtggctacacccaaaatggatccttcggccagtacatgctggtggatacccgatacgccgctcgcatcccagacggcgtggactacctcgaagcagcgccaattctgtgtgcaggcgtgactgtctacaaggcactcaaagtctctgaaacccgcccgggccaattcatggtgatctccggtgtcggcggacttggccacatcgcagtccaatacgcagcggcgatgggcatgcgtgtcattgcggtagatattgccgaggacaagctggaacttgcccgtaagcacggtgcggaatttaccgtgaatgcgcgtaatgaagatccaggcgaagctgtacagaagtacaccaacggtggcgcacacggcgtgcttgtgactgcagttcacgaggcagcattcggccaggcactggatatggctcgacgtgcaggaacaattgtgttcaacggtctgccaccgggagagttcccagcatccgtgttcaacatcgtattcaagggcctgaccatccgtggatccctcgtgggaacccgccaagacttggccgaagcgctcgatttctttgcacgcggactaatcaagccaaccgtgagtgagtgctccctcgatgaggtcaatggagttcttgaccgcatgcgaaacggcaagatcgatggtcgtgtggcgattcgtttctaa

SEQ ID NO: 44 - protein, 348 aa, Corynebacterium glutamicum
MSFMTTAAPQEFTAAVVEKFGHDVTVKDIDLPKPGPHQALVKVLTSGICHTDLHALEGDWPVKPEPPFVPGHEGVGEVVELGPGEHDVKVGDIVGNAWLWSACGTCEYCITGRETQCNEAEYGGYTQNGSFGQYMLVDTRYAARIPDGVDYLEAAPILCAGVTVYKALKVSETRPGQFMVISGVGGLGHIAVQYAAAMGMRVIAVDIAEDKLELARKHGAEFTVNARNEDPGEAVQKYTNGGAHGVLVTAVHEAAFGQALDMARRAGTIVFNGLPPGEFPASVFNIVFKGLTIRGSLVGTRQDLAEALDFFARGLIKPTVSECSLDEVNGVLDRMRNGKIDGRVAIRF

SEQ ID NO: 45 - DNA, 1020 bp, Corynebacterium glutamicum
atgcccaaatacattgccatgcaggtatccgaatccggtgcaccgttagccgcgaatctcgtgcaacctgctccgttgaaatcgagggaagtccgcgtggaaatcgctgctagtggtgtgtgccatgcagatattggcacggcagcagcatcggggaagcacactgtttttcctgttacccctggtcatgagattgcaggaaccatcgcggaaattggtgaaaacgtatctcggtggacggttggtgatcgcgttgcaatcggttggtttggtggcaattgcggtgactgcgctttttgtcgtgcaggtgatcctgtgcattgcagagagcggaagattcctggcgtttcttatgcgggtggttgggcacagaatattgttgttccagcggaggctcttgctgcgattccagatggcatggacttttacgaggccgccccgatgggctgcgcaggtgtgacaacattcaatgcgttgcgaaacctgaagctggatcccggtgcggctgtcgcggtctttggaatcggcggtttagtgcgcctagctattcagtttgctgcgaaaatgggttatcgaaccatcaccatcgcccgcggtttagagcgtgaggagctagctaggcaacttggcgccaaccactacatcgatagcaatgatctgcaccctggccaggcgttatttgaacttggcggggctgacttgatcttgtctactgcgtccaccacggagcctctttcggagttgtctaccggtctttctattggcgggcagctaaccattatcggagttgatgggggagatatcaccgtttcggcagcccaattgatgatgaaccgtcagatcatcacaggtcacctcactggaagtgcgaatgacacggaacagactatgaaatttgctcatctccatggcgtgaaaccgcttattgaacggatgcctctcgatcaagccaacgaggctattgcacgtatttcagctggtaaaccacgtttccgtattgtcttggagccgaattcataa

SEQ ID NO: 46 - protein, 339 aa, Corynebacterium glutamicum
MPKYIAMQVSESGAPLAANLVQPAPLKSREVRVEIAASGVCHADIGTAAASGKHTVFPVTPGHEIAGTIAEIGENVSRWTVGDRVAIGWFGGNCGDCAFCRAGDPVHCRERKIPGVSYAGGWAQNIVVPAEALAAIPDGMDFYEAAPMGCAGVTTFNALRNLKLDPGAAVAVFGIGGLVRLAIQFAAKMGYRTITIARGLEREELARQLGANHYIDSNDLHPGQALFELGGADLILSTASTTEPLSELSTGLSIGGQLTIIGVDGGDITVSAAQLMMNRQIITGHLTGSANDTEQTMKFAHLHGVKPLIERMPLDQANEAIARISAGKPRFRIVLEPNS

SEQ ID NO: 47 - DNA, 879 bp, Corynebacterium glutamicum
atgcaaacccttgctgctattgttcgtgccacgaagcaaccttttgagatcaccaccattgatctggatgcaccacgaccagatgaagttcaaatccgtgttattgctgccggagtgcgccacactgacgcaattgttcgtgatcagatttacccaacttttcttcccgcagttttcggccacgaaggcgccggagtagttgtcgccgtgggttctgcagtcacctcggtgaaaccagatgacaaggtagtgctgggattcaactcttgtggccagtgcttgaagtgtttgggcggtaagcctgcgtactgtgagaaattctatgaccgcaacttcgcatgcacccgcgatgccgggcacactactttgtttacccgtgcaacaaaagagcaggcagaggccatcatcgacacccttgatgatgttttctacgatgcggatgcgggtttcctggcatacccagcaactcccccagaggcttcgggagtaagcgtgttggttgtcgcggctggtacctctgatctcccccaagcaaaggaagcactacacactgcctcctacttggggcgctccacctcactgattgttgattttggagtggctggcatccaccgcctgctttcatacgaagaagaactccgcgctgcgggcgtgctcatcgttgccgctggaatggatggtgcgctacccggagttgtcgcaggcttagtgtccgcacctgtcgtcgcactgccaacctccgtgggatacggcgcaggtgctggaggaatcgcaccacttctgaccatgcttaacgcctgcgcgccgggagttggagtggtcaacattgataacggctatggagcaggacacctggctgcgcagattgcggcgaggtaa

SEQ ID NO: 48 - protein, 292 aa, Corynebacterium glutamicum
MQTLAAIVRATKQPFEITTIDLDAPRPDEVQIRVIAAGVRHTDAIVRDQIYPTFLPAVFGHEGAGVVVAVGSAVTSVKPDDKVVLGFNSCGQCLKCLGGKPAYCEKFYDRNFACTRDAGHTTLFTRATKEQAEAIIDTLDDVFYDADAGFLAYPATPPEASGVSVLVVAAGTSDLPQAKEALHTASYLGRSTSLIVDFGVAGIHRLLSYEEELRAAGVLIVAAGMDGALPGVVAGLVSAPVVALPTSVGYGAGAGGIAPLLTMLNACAPGVGVVNIDNGYGAGHLAAQIAAR

SEQ ID NO: 49 - DNA, 819 bp, Escherichia coli
atggaaacctatgctgtttttggtaatccgatagcccacagcaaatcgccattcattcatcagcaatttgctcagcaactgaatattgaacatccctatgggcgcgtgttggcacccatcaatgatttcatcaacacactgaacgctttctttagtgctggtggtaaaggtgcgaatgtgacggtgccttttaaagaagaggcttttgccagagcggatgagcttactgaacgggcagcgttggctggtgctgttaataccctcatgcggttagaagatggacgcctgctgggtgacaataccgatggtgtaggcttgttaagcgatctggaacgtctgtcttttatccgccctggtttacgtattctgcttatcggcgctggtggagcatctcgcggcgtactactgccactcctttccctggactgtgcggtgacaataactaatcggacggtatcccgcgcggaagagttggctaaattgtttgcgcacactggcagtattcaggcgttgagtatggacgaactggaaggtcatgagtttgatctcattattaatgcaacatccagtggcatcagtggtgatattccggcgatcccgtcatcgctcattcatccaggcatttattgctatgacatgttctatcagaaaggaaaaactccttttctggcatggtgtgagcagcgaggctcaaagcgtaatgctgatggtttaggaatgctggtggcacaggcggctcatgcctttcttctctggcacggtgttctgcctgacgtagaaccagttataaagcaattgcaggaggaattgtccgcgtga

SEQ ID NO: 50 - protein, 272 aa, Escherichia coli
METYAVFGNPIAHSKSPFIHQQFAQQLNIEHPYGRVLAPINDFINTLNAFFSAGGKGANVTVPFKEEAFARADELTERAALAGAVNTLMRLEDGRLLGDNTDGVGLLSDLERLSFIRPGLRILLIGAGGASRGVLLPLLSLDCAVTITNRTVSRAEELAKLFAHTGSIQALSMDELEGHEFDLIINATSSGISGDIPAIPSSLIHPGIYCYDMFYQKGKTPFLAWCEQRGSKRNADGLGMLVAQAAHAFLLWHGVLPDVEPVIKQLQEELSA

SEQ ID NO: 51 - DNA, 35 bp, Artificial Sequence
  primer
cggtacccggggatccttacttccgcgtatccaac

SEQ ID NO: 52 - DNA, 41 bp, Artificial Sequence
  primer
ctaggaatcgcggccggtgaactcctaaagaactatataac

SEQ ID NO: 53 - DNA, 20 bp, Artificial Sequence
  primer
ggccgcgattcctagcatgc

SEQ ID NO: 54 - DNA, 35 bp, Artificial Sequence
  primer
ccaagcttgcatgccagtcatcatcaacggtgccg

SEQ ID NO: 55 - DNA, 21 bp, Artificial Sequence
  primer
atctccgcagaagacgtactg

SEQ ID NO: 56 - DNA, 20 bp, Artificial Sequence
  primer
tccgatcatgtatgacctcc

SEQ ID NO: 57 - DNA, 36 bp, Artificial Sequence
  primer
cggtacccggggatcggcatagtgcttccaacgctc

SEQ ID NO: 58 - DNA, 36 bp, Artificial Sequence
  primer
tagctccactcaagattcctcgatattacctacagg

SEQ ID NO: 59 - DNA, 20 bp, Artificial Sequence
  primer
tcttgagtggagctagggcc

SEQ ID NO: 60 - DNA, 37 bp, Artificial Sequence
  primer
ccaagcttgcatgcccatatagagcccaggagctctc

SEQ ID NO: 61 - DNA, 23 bp, Artificial Sequence
  primer
cgccgcaaagtccaaatagaaag

SEQ ID NO: 62 - DNA, 20 bp, Artificial Sequence
  primer
ggattcttcctgaactcagc

SEQ ID NO: 63 - DNA, 36 bp, Artificial Sequence
  primer
cggtacccggggatcgggctcgtcctgaaattgcac

SEQ ID NO: 64 - DNA, 35 bp, Artificial Sequence
  primer
tccgtcgtgagccatgttgtgcccacgagactacc

SEQ ID NO: 65 - DNA, 20 bp, Artificial Sequence
  primer
atggctcacgacggattgcg

SEQ ID NO: 66 - DNA, 36 bp, Artificial Sequence
  primer
ccaagcttgcatgcccggttgcagccttcataaacg

SEQ ID NO: 67 - DNA, 21 bp, Artificial Sequence
  primer
agaccaatgagtacccaaccg

SEQ ID NO: 68 - DNA, 20 bp, Artificial Sequence
  primer
tcagcgtctggctcagctac

SEQ ID NO: 69 - DNA, 36 bp, Artificial Sequence
  primer
cggtacccggggatcaaccccagctcaaataacacc

SEQ ID NO: 70 - DNA, 37 bp, Artificial Sequence
  primer
tttcaacacaatccgtccttctcgcttggattacttg

SEQ ID NO: 71 - DNA, 23 bp, Artificial Sequence
  primer
cggattgtgttgaaattgctctg

SEQ ID NO: 72 - DNA, 35 bp, Artificial Sequence
  primer
ccaagcttgcatgcctcaccacgggaatcttcagg

SEQ ID NO: 73 - DNA, 20 bp, Artificial Sequence
  primer
ccggactggggtgtgttttg

SEQ ID NO: 74 - DNA, 20 bp, Artificial Sequence
  primer
cccggaaaatacggtatagc

SEQ ID NO: 75 - DNA, 47 bp, Artificial Sequence
  primer
ccaagcttgcatgccaggaggattataatgcgcctgcgtgtctcgag

SEQ ID NO: 76 - DNA, 34 bp, Artificial Sequence
  primer
cggtacccggggatccaactacgcggcgacgtac

SEQ ID NO: 77 - DNA, 3387 bp, Gordonia effusa
atgagcgatcagccgaatgcactgccgagcgcaattgaaccgctgaatccggatccgcaggcaaccgagcagattagccattgtgcaaccattgcagaactggttcgtgttctggcagaaagctatggtgatcgtccggcactgggttggcgtaataatagcgatccgagcagctggcatagcatgacctatcgtgatctggccgaacgtgcagatagcatggcacgtctgctgcatagcaccctgggtgttgcagaaaatgatcgtgttgcaaccgttggttttaccagcgcagaatataccattgcaagcctggcagttggtacactgggtgcaatggaagttccgctgcagaatgcaggtagcgttgatgtttgggcagcaattctgaccgaaaccgattgtgttagcgcagttgttgcagcagatcagctgccgagcattgcccgtctggcggaaagcggcacctataccggtctgcgtcatgttctggtttttgatattggtagccgtgatggcaccaccctggatgatgcagcacgtcgtctggttgccgcaggcacccaggttcatctgcgtcagcctggtgcagaaccgaccacccctccggcaccgctgccgcagattaccgcaaacccggatcgtgtggcactgctgatttataccagcggtagcacaggtgcaccgaaaggtgcaatgtataccgaaacagcagttacccgtctgtttcagagcggtctgagtggtctgggtcgtgcaaccgatggtcatggttggattaccctgaactttatgccgatgagccatgttatgggtcgtagtaccctgtggcagaccctgggtaatggtggcaccgcatattttacaccgcgtgcagatctggctgaactgctgaccgatctggcagccgttcagccgacggatctgcagtttgttccgcgtatttgggatatgctgtatcaagaatatgttcgtctgacagatcaggatgttagcgaacaggatgcactgacccgtatgcgtgaacattatttcggcacccgtaccgcaaccgcaattaccggtagcgcaccgattagtgatgaagttcgtcgttttgttgaagcaatgctgccggttccgctgattgaaggttatggtagcaccgaagcagccggtgttagcattgatggtcgtattcagcgtccgcctgttgttgattataaactgctggatgtgccggaactgggttatctgagcaccgatcgtccgcatccgcgtggtgagctgctggttaaaaccgatcatatttttgccggttattacaatcgtccggatctgaccagcagcgtttttgatgatcagggttattatcgtaccggtgatattgttgccgaaaccggtccggatcagattgaatatgttgatcgtcgtaacaacgtgatgaaactgagccagggtgaatttgttgcaattgcccatattgaagcagttctgaccaccccaccgattcagcagctgtatgtttatggtaatagcgcacgtccgtatctgctggccgttgttgttccgacaccggaactgcgtgaacgtcatgcagatgataatgaactgcgtcgtgaagttctgacagcactgcgtagccatggtgaacgtaatggtctggcagcagttgaaattccgcgtgatgttattgttgaacgtaccccgtttagcctggaaaatggtctgctgacaggtattcgtaaactggcacgtccgcagctgaaagaacgttatggtgcacgtctggaagcactgtatgccgaactggccgatagccgtattacacgtctgcgtgatgtgaaagcagttgcagcccagcgtagcaccgttaccaccgttattgatgttgttaccgcaattctggatctggcggatggtgaagttaccgcagcagcacattttacagatctgggtggtgatagcctgaccgcagttaccgttggtaacgaactgcgcgatatttttgatgccgaagttccggttggtgtgctgaccagcccgagcagtaccctggcagatattgcggaacatattgatggccgtcatagcgaagcacgtccgaccgcagaaagcgttcatggcaccggtacaaccctgcgtgcagccgatctgaccctggataaatttctggatgaagaaacactgcgtgccgcaagtgatgttaccagtgcagccaccgatgttcgtaccgtgtttattaccggtgcaaccggttttctgggtcgctacctgacactggattggctgcgtcgtatggcaaaagttggtggtacagttatttgtctggtgcgtggtgccgatgatgacgcagcccgtgcgcgtctggatgcagcatttgatagcagcgatctgtggtctgaatatcagcgtctggcaaaagatcatctgcgcgtgctggcaggcgataaagatagcgatcatctggcactgacaccggatgtgtgggatgaactggcaaaaagcgttgatctgattattgatccggcagcactggttaatcatgtactgccgtatcgcgaactgtttggtccgaatgttagcggcaccgcagaactgatccgtctggcagttaccaccacccgtaaaccgtatgtgtatatttcaaccgtgggtgttggtgatcaggttgctccgggtagctttaccgaagatcctgatattcgtgaaatgagcagcgtgcgtgaaatcaatgatacctatgcaaatggttacggcaatagcaaatgggcaggcgaagttctgctggcacaggcacatgaacgttttgaactgccggttagcgtttttcgttgtgatatgattgttgcggatgatcataccattggtcagctgaatctgccggatatgtttactcgcctgctgatgagcgttctggcaacaggtctggcaccgcgtagcttttatcagctggcgaccgatggtagtgcacaagaggcacattttgatgcgctgccggtggatttcctggccgaagcaattaatacactgtgggttaaagatggtgcccgtacctttaatgcaatgaatccgcatgccgatggtattggttttgatcagtatattcgttggctgattgatagcggtgaacaaattagcctggtggataattatgatgattggtatcgtcgctttggtgccgcactggcggatctgcctgaaaaacagcgtcgtggtagcctgattccgctgctgcacaattatgttcatccgatgacaccgcataatcgtggtatggcaagcgcagatcgttttcatgatgcagttcgtacagcaggcgttggtcagagcagcgatattccgcatattacccctcagattattgaaaattatgcacgtagcctgcgtggcctgggtgtgatttaa

SEQ ID NO: 78 - DNA, 3408 bp, Novosphingobium malaysiense
atggatgccgagagcggagtcatgccgagcgatcccgatgtggttgccttcgtccgccggccggacacgtgccttagcgcgatgatcgagaaagcgctcgattcctatgccgggcgcgatgcattagcctggcgccccacgcgttcaggcgtgttgagcgataccttcgaagtcatgacctacaaggacctggcaaggcgcgtccgctccgtggcgacggcgctcgccaaagaccccgatctgggtctgaaagccggcgacccgatcgggatcatggcctttgccaacgtcgacttcgtcaccctcaatctcgcgctgggcctctgcggtggcgttatcgcgccgctgcagacctccgccagcatggaagcactgaccgggctggtcagggaactggcagcgccctgcctcgccgcatcgctcgaacatctcgaagcgatcaccacgctcgccatcgcaagcgaaaaaacgcgcgcaatccttatcttcgaccacgatggcctcgacgaagatgcccgggccgcgatcgccgccgcccagcaacgcctagacgcggaaaagcccggctgcctgatcctgccgttttccgaagtgatcgcacgcggcgaaaagctgccgccgctcgatcccttcgttccggcgccgggcgaggaccccttggctctgatctattacacctcgggcagcaccggcacaccaaagggcgttatgtacacgcagaagctggtgaagctgggctattcgatagcccgcgaccatgccccgatcgtcctgcactatcagccgctcaaccactccttcgggatgtccttcatcgccatggccctcgccagcggcggcacgtcctactttaccgccaagagcgacctgtcgacgctgctgagcgacatgaagatggtccgcccgacgaccatggctctcgtcccgcgcatatcggaaatgctgttccagcgtttccatgccgactacgccgacgagatcgcacgcgacgaggatgccgcaatggcgcggttccgcgaagacgttctcggggggcggatgaccgacatcgtcaccggggccgcacctacttcgccggaacttcgcgacttcatcgagaagatgaccggtctcacactgatggaagggtacggctgcaccgaagcaggcggctcgatcaccttcaacgaccgggtgatgcgcccgcccgtgctcgaataccgcctgatcgacgtgcccgagctcggctatttcactaccgatacgccccatccgcgcggcgagctcatcctcaagagcgatgcgatgttcgccgggtacttcgcgcgtccggacctcacggcaaaggccttcgacgacgaggggttctaccataccggcgacattatggccgagatcgaacccgaccacctcgtctacctcgaccgcaccaacaacgtgatgaagctgtcgcagggcgaattcgtaccggtcgcgttgctggaatcgctctatgcgggcggtgatccggtgatccgccagatctatctctatggcaattcgacgcgggctttcctgctcggcgtggccgtgcccaacatggatgccctgcccgagggaatcggtgatgaggaaatcaaggcccgcatgctccaggctctggaacgcatcgccagggccaacgaacgccattcctacgaagtcccgcgcgacctgattatagagcatgagccgttctctcccgaaaacggcctgcttgcgggcgtcggcaagtacatgcgccccgccttcaaggcgcgatacggagagcagctcgaagcgctctatgaagaaatcgctcgcagtcaggaccgcgagctgcaggaattgcgcagaaccggccgcaccttcccagttctcgaaaccgtgtgccgggcggccggcgccgtactgggcggcaagaccgttgccctttccgagacaggctccttcgcgtcgtcgggtggggattcgctttcagcactgtccctctcgctgcttttggaggacatctacgaactgcccgtcgaagtcagcgcgatcctccatccctcgggcacgtacgggctgcttgccgcggaaatcgaggagaagctgggcggcggtgcgaagcgacgcgacgccgtggccgttcatggcgcggacctcaccgtgctcaaggcggccgacctgacgctcgacaagttcatagacgccgagatccttggcgccgccaccggcctgcccgcgccgcccgacgctgaaccagaggtggtgcttctcaccggtgtcaccggcttcctaggccgtttcatgtgcctggaatggctgcgtcggctggagcgcaacggcaagggcaaggtggtctgcgtggcgcgcggtgccgatgacgacgatgcccgccgccgcgtcctggcaggctttgaaggcggtgatggcgcactggcggcggaagtggcccggctgggcgaaggccggctggccgtcttcgcaggcgatcttgccgcaccccggctgggtctcaccgcgacatgctggcaggcgctgtgcgaccaggtggacctcattgctcaccctggcgccttcgtgaaccacaagctgccctaccgccagctgttcggagccaacacagcaggcacggccgaactgatcgcgctggctctcaccacgcgcaagaagcgcttcgcccatgtctctaccatcgccacgacatacaacgatggtcatcgcgcggatgaaaacggctacatcgacagcgccattcccgaatggcatgtaagcgacgcctacgccgacggctatgggtcgtccaaatgggccgcagaagtgctgctggccagagccaatgagcaatatggcctacccgtttcggtctaccgttcgaacatgatcatggcacccggcgagttctccggtcagctcaatgtgcccgatatcttcactcgcctgctgctgagcctggcgctgacccggctggcccccgccagcttctattcgggcgattccgcgcgggcccattacgaaggcctgccggtcgatttcctggcccgcgccatcgtgaccattgccgaagacaaccgcgcggggttccataccttccacacgatcaacccgcacgatgacgggatctcgaccgacactttcgtcgactggatcggtgaagcgggcattccgatcgaacggatcgcggactacgacgaatgggtcacgcgtttcgggacggccctgcgcgccctgcctgaaaagcagcggcaagcctcgatcctgccgttgatggacgcgtacaagcacccgtccccggcgatccccgacttccgcgatcaggcacctaacttccgccaggcggttgccgaatcgcaagtgaacggagacggcgcgatccctcatctcacgccggcattgattgctcggtatctggaggacctgaaggccaccggcctgctcacctcctga

SEQ ID NO: 79 - protein, 1135 aa, Novosphingobium malaysiense
MDAESGVMPSDPDVVAFVRRPDTCLSAMIEKALDSYAGRDALAWRPTRSGVLSDTFEVMTYKDLARRVRSVATALAKDPDLGLKAGDPIGIMAFANVDFVTLNLALGLCGGVIAPLQTSASMEALTGLVRELAAPCLAASLEHLEAITTLAIASEKTRAILIFDHDGLDEDARAAIAAAQQRLDAEKPGCLILPFSEVIARGEKLPPLDPFVPAPGEDPLALIYYTSGSTGTPKGVMYTQKLVKLGYSIARDHAPIVLHYQPLNHSFGMSFIAMALASGGTSYFTAKSDLSTLLSDMKMVRPTTMALVPRISEMLFQRFHADYADEIARDEDAAMARFREDVLGGRMTDIVTGAAPTSPELRDFIEKMTGLTLMEGYGCTEAGGSITFNDRVMRPPVLEYRLIDVPELGYFTTDTPHPRGELILKSDAMFAGYFARPDLTAKAFDDEGFYHTGDIMAEIEPDHLVYLDRTNNVMKLSQGEFVPVALLESLYAGGDPVIRQIYLYGNSTRAFLLGVAVPNMDALPEGIGDEEIKARMLQALERIARANERHSYEVPRDLIIEHEPFSPENGLLAGVGKYMRPAFKARYGEQLEALYEEIARSQDRELQELRRTGRTFPVLETVCRAAGAVLGGKTVALSETGSFASSGGDSLSALSLSLLLEDIYELPVEVSAILHPSGTYGLLAAEIEEKLGGGAKRRDAVAVHGADLTVLKAADLTLDKFIDAEILGAATGLPAPPDAEPEVVLLTGVTGFLGRFMCLEWLRRLERNGKGKVVCVARGADDDDARRRVLAGFEGGDGALAAEVARLGEGRLAVFAGDLAAPRLGLTATCWQALCDQVDLIAHPGAFVNHKLPYRQLFGANTAGTAELIALALTTRKKRFAHVSTIATTYNDGHRADENGYIDSAIPEWHVSDAYADGYGSSKWAAEVLLARANEQYGLPVSVYRSNMIMAPGEFSGQLNVPDIFTRLLLSLALTRLAPASFYSGDSARAHYEGLPVDFLARAIVTIAEDNRAGFHTFHTINPHDDGISTDTFVDWIGEAGIPIERIADYDEWVTRFGTALRALPEKQRQASILPLMDAYKHPSPAIPDFRDQAPNFRQAVAESQVNGDGAIPHLTPALIARYLEDLKATGLLTS

SEQ ID NO: 80 - DNA, 4543 bp, Artificial Sequence
  Nucleotide sequence of DNA fragment containing ACAR gene of Novosphingobium malaysiense (codon-optimized) and entD gene of Escherichia coli
ccaagcttgcatgccagatcgtttagatccgaaggaaaacgtcgaaaagcaatttgcttttcgacgccccaccccgcgcgttttagcgtgtcagtagacgcgtagggtaagtggggtagcggcttgttagatatcttgaaatcggctttcaacagcattgatttcgatgtatttagctggccgtttgagacgcgatgtccacagggtagctggtagtttgaaaatcaacgccgttgcccttaggattcagtaactggcacattttgtaatgcgctagatctgtgtgcccagtcttccaggctgcttatcacagtgaaagcaaaaccaattcgtggctgcgaaagtcgtagccaccacgaagtccaggaggacatacaatggatgcagaaagcggtgttatgccgagcgatccggatgttgttgcatttgttcgtcgtccggatacctgtctgagcgcaatgattgaaaaagcactggatagctatgcaggtcgtgatgcactggcatggcgtccgacccgtagcggtgttctgagcgatacctttgaagttatgacctataaagatctggcacgtcgtgttcgtagcgttgcaaccgcactggcaaaagatcctgatctgggtctgaaagccggtgatccgattggtattatggcatttgccaatgttgatttcgttaccctgaatctggcactgggtctgtgtggtggtgttattgcaccgctgcagaccagcgcaagcatggaagcactgaccggtctggttcgtgaactggcagcaccgtgtctggcagcaagcctggaacatctggaagcaattaccaccctggcaattgcaagcgaaaaaacccgtgcaattctgatctttgatcatgatggtctggatgaagatgcacgtgccgcaattgcagcagcacagcagcgtctggatgccgaaaaaccgggttgtctgattctgccgtttagcgaagttattgcccgtggtgaaaaactgcctccgctggatccgtttgttccggcaccgggtgaagatccgctggcactgatctattataccagcggtagcaccggcaccccgaaaggtgttatgtatacccagaaactggttaaactgggttatagcattgcacgtgatcatgcaccgattgttctgcattatcagccgctgaatcatagctttggtatgagctttattgcaatggcactggcgagcggtggcaccagctattttaccgcaaaaagcgatctgagcaccctgctgagtgatatgaaaatggttcgtccgaccaccatggccctggttccgcgtattagcgaaatgctgtttcagcgttttcatgcagattatgcagatgaaattgcgcgtgatgaggatgcagccatggcacgttttcgtgaagatgttctgggtggtcgtatgaccgatattgttaccggtgcagcaccgaccagtccggaactgcgtgattttattgaaaaaatgacaggtctgaccctgatggaaggttatggttgtaccgaagccggtggtagcattacctttaatgatcgtgttatgcgtccgcctgttctggaatatcgtctgattgatgttcctgaactgggatattttaccaccgatacaccgcatccgcgtggtgaactgattctgaaaagtgatgcaatgtttgccggttattttgcacgtccggatctgaccgcaaaagcatttgatgatgaaggcttttatcacaccggtgatattatggccgaaattgaaccggatcatctggtttatctggatcgtaccaataacgtgatgaaactgagccagggtgaatttgtgccggttgcactgctggaaagcctgtatgccggtggtgatccggtgattcgtcagatttatctgtatggtaatagcacccgtgcctttctgctgggtgttgcagttccgaatatggatgcactgccggaaggtattggtgatgaagaaattaaagcacgtatgctgcaggcactggaacgtattgcacgcgcaaatgaacgtcatagttatgaagttccgcgtgatctgattattgaacacgaaccgtttagtccggaaaatggtctgctggcaggcgttggcaaatatatgcgtcctgcatttaaagcccgttatggtgagcagctggaagccctgtacgaagaaattgcacgtagccaggatcgcgaactgcaagaactgcgtcgtaccggtcgtacctttccggttctggaaaccgtttgtcgtgcagccggtgcagtgctgggtggcaaaaccgttgcactgagcgaaaccggtagctttgcaagcagtggtggtgatagcctgagcgcactgagcctgagcctgctgctggaagatatttatgaactgccggttgaagttagcgcaatcctgcatccgagcggcacctacggcctgctggctgcagaaattgaagaaaaactgggtggtggtgcaaaacgccgtgatgcagttgccgttcatggtgcagatctgacagttctgaaagcagccgatctgacactggataaattcattgatgcggaaattctgggtgcagcaaccggtctgcctgcccctcctgatgccgaaccggaagttgttctgctgaccggtgttacaggttttctgggtcgttttatgtgtctggaatggctgcgtcgtctggaacgcaatggtaaaggtaaagttgtttgtgttgcacgtggtgccgatgatgatgacgcacgtcgtcgcgttctggcaggttttgaaggtggtgatggtgccctggcagccgaagttgcacgtctgggtgaaggtcgtctggccgtttttgcgggtgatctggcagcccctcgtctgggcctgaccgccacatgttggcaggccctgtgtgatcaggtggatctgattgcacatccgggtgcctttgttaatcataaactgccgtatcgtcagctgtttggtgcaaataccgcaggcaccgcagaactgattgccctggccctgaccacccgtaaaaaacgctttgcacatgttagcaccattgccaccacctataatgatggtcatcgtgcggatgaaaacggctatattgatagcgccatcccggaatggcatgttagtgatgcatatgccgatggttatggtagctcaaaatgggcagcggaagtgctgctggcacgtgcgaatgaacagtatggtctgccggtgagcgtttatcgtagcaatatgattatggcacctggtgaatttagcggtcagctgaatgttccggatatctttacccgtctgctgctgagcctggcgctgacccgtctggcaccggcaagcttttatagcggtgatagcgcacgtgcacattatgaaggcctgccggtggattttctggctcgtgccattgtgaccattgccgaagataatcgtgcaggttttcatacctttcacaccattaatccgcatgatgatggtattagcacagatacatttgtggattggattggtgaagcaggtattccgattgaacgcattgcggattatgatgaatgggttacccgttttggcaccgcactgcgtgccctgccggaaaaacagcgtcaggcaagcattctgccgctgatggatgcatataaacatccgagtccggcaattccggattttcgcgatcaggcaccgaattttcgtcaggcagttgcggaaagccaggttaatggtgatggcgcaattccgcatctgacaccggcactgattgcgcgttatctggaagatctgaaagcgacaggcctgctgaccagctaaaggaggacatacaatggtcgatatgaaaactacgcatacctccctcccctttgccggacatacgctgcattttgttgagttcgatccggcgaatttttgtgagcaggatttactctggctgccgcactacgcacaactgcaacacgctggacgtaaacgtaaaacagagcatttagccggacggatcgctgctgtttatgctttgcgggaatatggctataaatgtgtgcccgcaatcggcgagctacgccaacctgtctggcctgcggaggtatacggcagtattagccactgtgggactacggcattagccgtggtatctcgtcaaccgattggcattgatatagaagaaattttttctgtacaaaccgcaagagaattgacagacaacattattacaccagcggaacacgagcgactcgcagactgcggtttagccttttctctggcgctgacactggcattttccgccaaagagagcgcatttaaggcaagtgagatccaaactgatgcaggttttctggactatcagataattagctggaataaacagcaggtcatcattcatcgtgagaatgagatgtttgctgtgcactggcagataaaagaaaagatagtcataacgctgtgccaacacgattaattgacaacatctggtacgattcgcccgcagccatcactgaccacgggcgaaagtgtaaagcaggtgccttaccatcctgacctgacaaccggatatgcgggatccccgggtaccg

SEQ ID NO: 81 - DNA, 3408 bp, Novosphingobium malaysiense
atggatgcagaaagcggtgttatgccgagcgatccggatgttgttgcatttgttcgtcgtccggatacctgtctgagcgcaatgattgaaaaagcactggatagctatgcaggtcgtgatgcactggcatggcgtccgacccgtagcggtgttctgagcgatacctttgaagttatgacctataaagatctggcacgtcgtgttcgtagcgttgcaaccgcactggcaaaagatcctgatctgggtctgaaagccggtgatccgattggtattatggcatttgccaatgttgatttcgttaccctgaatctggcactgggtctgtgtggtggtgttattgcaccgctgcagaccagcgcaagcatggaagcactgaccggtctggttcgtgaactggcagcaccgtgtctggcagcaagcctggaacatctggaagcaattaccaccctggcaattgcaagcgaaaaaacccgtgcaattctgatctttgatcatgatggtctggatgaagatgcacgtgccgcaattgcagcagcacagcagcgtctggatgccgaaaaaccgggttgtctgattctgccgtttagcgaagttattgcccgtggtgaaaaactgcctccgctggatccgtttgttccggcaccgggtgaagatccgctggcactgatctattataccagcggtagcaccggcaccccgaaaggtgttatgtatacccagaaactggttaaactgggttatagcattgcacgtgatcatgcaccgattgttctgcattatcagccgctgaatcatagctttggtatgagctttattgcaatggcactggcgagcggtggcaccagctattttaccgcaaaaagcgatctgagcaccctgctgagtgatatgaaaatggttcgtccgaccaccatggccctggttccgcgtattagcgaaatgctgtttcagcgttttcatgcagattatgcagatgaaattgcgcgtgatgaggatgcagccatggcacgttttcgtgaagatgttctgggtggtcgtatgaccgatattgttaccggtgcagcaccgaccagtccggaactgcgtgattttattgaaaaaatgacaggtctgaccctgatggaaggttatggttgtaccgaagccggtggtagcattacctttaatgatcgtgttatgcgtccgcctgttctggaatatcgtctgattgatgttcctgaactgggatattttaccaccgatacaccgcatccgcgtggtgaactgattctgaaaagtgatgcaatgtttgccggttattttgcacgtccggatctgaccgcaaaagcatttgatgatgaaggcttttatcacaccggtgatattatggccgaaattgaaccggatcatctggtttatctggatcgtaccaataacgtgatgaaactgagccagggtgaatttgtgccggttgcactgctggaaagcctgtatgccggtggtgatccggtgattcgtcagatttatctgtatggtaatagcacccgtgcctttctgctgggtgttgcagttccgaatatggatgcactgccggaaggtattggtgatgaagaaattaaagcacgtatgctgcaggcactggaacgtattgcacgcgcaaatgaacgtcatagttatgaagttccgcgtgatctgattattgaacacgaaccgtttagtccggaaaatggtctgctggcaggcgttggcaaatatatgcgtcctgcatttaaagcccgttatggtgagcagctggaagccctgtacgaagaaattgcacgtagccaggatcgcgaactgcaagaactgcgtcgtaccggtcgtacctttccggttctggaaaccgtttgtcgtgcagccggtgcagtgctgggtggcaaaaccgttgcactgagcgaaaccggtagctttgcaagcagtggtggtgatagcctgagcgcactgagcctgagcctgctgctggaagatatttatgaactgccggttgaagttagcgcaatcctgcatccgagcggcacctacggcctgctggctgcagaaattgaagaaaaactgggtggtggtgcaaaacgccgtgatgcagttgccgttcatggtgcagatctgacagttctgaaagcagccgatctgacactggataaattcattgatgcggaaattctgggtgcagcaaccggtctgcctgcccctcctgatgccgaaccggaagttgttctgctgaccggtgttacaggttttctgggtcgttttatgtgtctggaatggctgcgtcgtctggaacgcaatggtaaaggtaaagttgtttgtgttgcacgtggtgccgatgatgatgacgcacgtcgtcgcgttctggcaggttttgaaggtggtgatggtgccctggcagccgaagttgcacgtctgggtgaaggtcgtctggccgtttttgcgggtgatctggcagcccctcgtctgggcctgaccgccacatgttggcaggccctgtgtgatcaggtggatctgattgcacatccgggtgcctttgttaatcataaactgccgtatcgtcagctgtttggtgcaaataccgcaggcaccgcagaactgattgccctggccctgaccacccgtaaaaaacgctttgcacatgttagcaccattgccaccacctataatgatggtcatcgtgcggatgaaaacggctatattgatagcgccatcccggaatggcatgttagtgatgcatatgccgatggttatggtagctcaaaatgggcagcggaagtgctgctggcacgtgcgaatgaacagtatggtctgccggtgagcgtttatcgtagcaatatgattatggcacctggtgaatttagcggtcagctgaatgttccggatatctttacccgtctgctgctgagcctggcgctgacccgtctggcaccggcaagcttttatagcggtgatagcgcacgtgcacattatgaaggcctgccggtggattttctggctcgtgccattgtgaccattgccgaagataatcgtgcaggttttcatacctttcacaccattaatccgcatgatgatggtattagcacagatacatttgtggattggattggtgaagcaggtattccgattgaacgcattgcggattatgatgaatgggttacccgttttggcaccgcactgcgtgccctgccggaaaaacagcgtcaggcaagcattctgccgctgatggatgcatataaacatccgagtccggcaattccggattttcgcgatcaggcaccgaattttcgtcaggcagttgcggaaagccaggttaatggtgatggcgcaattccgcatctgacaccggcactgattgcgcgttatctggaagatctgaaagcgacaggcctgctgaccagctaa

SEQ ID NO: 82 - DNA, 3582 bp, Coccomyxa subellipsoidea
atgacagagaacggaggactacctcaggtcaatggaggcggcccccagtactgggagatgtccaacggccagaaccagactaacaatgtcattcagaagaggcttgcccgcgctcgcgaagtcatcaagcaagacccccagctgcaggcggccaagtttgacaggaaatcacttcaacggatcacggatgcggggaacaccagcattgagattattgcggccatgttcaaggagtatgcgtcgcgcgatctattcggcgcctgcacaccgggagagtccaccttccacactgtgacttatggagcagtctgggagcgcattcaggcgctggtggcgggctggacagcgctgggattcgtggctccgggggactttgtggggatctctgggtttgccagcgtggactgggtggtgtctgatctggcgacgctgcatgctgggggggtcatggtccccctgcccacaaacatcctggcagaggacgtgcgcgcaatcattgacgaggctgaagtgcgttgcctcatggtcagcgctgaggagcttgcggccattgcaccggtcatcggcggctgcgcgagcgtgaaggccgtcattgtcatggacagttccacggacgccgtgacatcctcgggagcctacgcggagatgcaggccaacctgccggcaggcgcaaagctgaccaccatcgacgaagttttggcggcaggccgcgcaaccggcaagcagcccgcactggtgatccccggcagggatgggcggcccgcggaccccttagtaaacctcatgtacacctcgggcagctctgggcgtcccaagggggccgagtaccccgagcacctcatctttgacttcctcaagaactcgatgcccacagatgcgccggagctgccgaccatcataatgggcttccttcctttaaaccatttgatgggaagatttactctgctcaagtgcctgctcaccggaggccagaactggtttgtgcgctcgaccgacatgtcgaccttcttcgatgacctggcgacgatccgtcccacggaggcgatgttccctccgcggattatgaacatgctgcacgacagattcgtggagcagctcgaccgcctgccgccagcccccagcgaggccgagcgcgcgcagcaacgccaggacctgatcaagcgcttcagggaagtggacttgggtggccgcctcttcaccggctcctttggcagcgcgccagcgtccccagatgtgatccaatggctggaggaggtcctcggcttccccccagtgaatggctacggctccacagagggcggcatgatcatgctcgacaacaagatccagcatagttatgtgccggcgtacaagctggtagatgtgccagagctgggctacaccacaaaggacaagcccttcccccgcggagaactgcgcatcaagacccggcgcatgatcccgggctactacaaacatcctgaggcaacagcggatctgtttgacgaggagggcttcctgaagactggggatgtggtggagcagcgcgatgcagacaccttcatctggctggaccgcgtcaagaacatcatcaagctctcacagggtgagtacgtgagcgtgtcgcggctggaggagatctatgtgggcaactccaagctcatccaccagatgtacatctacgggaactccctccgtgcctacctggtcgccgtcgtcgtgccccacatcgagaacggagcgtgtgcggatgcgggcaagctgagggcggcgctgcggacagagctggatgacgtggcgcgacgcaaggcactacaggggtatgagatcccgcgcgagttcatagtggagatgcgccccttctccaaggacaatcacctgctcactgactccgccaagcccgcccgcggccagctcaagaagaggtaccaggcggagctggagggcctttacacggccctggaggagcgtctgcgcgagagactgcgcgccatgaaggagggcaaggatgcatctgtgcaggaccgtatcaagcaggcgctggaggttactctgggactggcggaggaggacatggcggacgtggcttcgcgcagcttcgcgcagctgggcggtgactcgctggcggcgatccagtttgcgcgctacgtgggcgagctttgcggcgtcaacctgccggtgtcctttgtgctggaccactcccactccctccaggccatcgccgaccgcgtccacgaactcgtcagcggcgacgcgagcgcagggatcacgttcgagtcgatccacggcagcgatggcgtgaacatcaaggcagccgacctgaagctggaccggttcctatcagaagctgacacggccgcggccgccgcggccgccccggcctccgagctgccggcgcggccgacacacgtgctgctgaccggcgccaacggcttcctcggccgcttcctgctgctggacctgctgcagcgcggttctgacaagaatggaggccgtgtggtggctatagtgcgcggcagcagcgatgagaaggcggctgagcggctgcgcgccggttttgacagcggtgacgcgaccctgctgcagcgctatgacaccctcagcaagcatctgaccgtctatgcaggcgacctggcgaagccgcagctgggcctgagccagggggtgtatgagtcgctgtgcgctgagctggacaccatcgtgcacaacggcgcgctggtcaaccacgcttactcctatgagcagctctttgagcccaatgtgctcggcagcgtggaggtgatgcggatggctctggcaaagcgcagaaaggcgctgacattcatctccagtgtgggagtggtgggaggcctggaccacccacagccggtgactgaggctgaggacggtccaactctgtgtgatgtgcacccgggcgacggcggctacgccatcgggtacggctgcagcaagtgggcggtggaggtgcttctcaaggagctgcaccagcgctggggtgttcccgtcaaggtcttccgctgcggcatgatcctgtcgcacaccagctacttgggccagatcaacccaaccgacttcttcacgcggctgctgtgcggcattgcctacacggggatcgccccgcagtccttctacaccctgccccacggccccgaggagcactttgacggcatgcccatcgacttcgtgtccggcgtgatctctgccacaacggcggccgagcgcagcggcttcgacacgtaccatgtggtcaatccccactggagcgacggcgtatccctcgaccgcatcgtcgactgggcggagagcgccggctacccggttaatcgcatcgcgccatatgagcagtggtacgcgcagttcaaggcagcgctggaggctcttgaccacacgcggcagcagcagtcgccgctgcccatcatctaccaatgggagcgcccggcatccggcaccagcggcacgaagtacgatgccacgcagctgcgcaagagggcggccgcatacacacagtggaaggacgtgccccatctggacgaggcgttcatccaccagaacatgcgccacctcaccaccctgcgcctcatcacccctcccggcaaggcctga

SEQ ID NO: 83 - protein, 1193 aa, Coccomyxa subellipsoidea
MTENGGLPQVNGGGPQYWEMSNGQNQTNNVIQKRLARAREVIKQDPQLQAAKFDRKSLQRITDAGNTSIEIIAAMFKEYASRDLFGACTPGESTFHTVTYGAVWERIQALVAGWTALGFVAPGDFVGISGFASVDWVVSDLATLHAGGVMVPLPTNILAEDVRAIIDEAEVRCLMVSAEELAAIAPVIGGCASVKAVIVMDSSTDAVTSSGAYAEMQANLPAGAKLTTIDEVLAAGRATGKQPALVIPGRDGRPADPLVNLMYTSGSSGRPKGAEYPEHLIFDFLKNSMPTDAPELPTIIMGFLPLNHLMGRFTLLKCLLTGGQNWFVRSTDMSTFFDDLATIRPTEAMFPPRIMNMLHDRFVEQLDRLPPAPSEAERAQQRQDLIKRFREVDLGGRLFTGSFGSAPASPDVIQWLEEVLGFPPVNGYGSTEGGMIMLDNKIQHSYVPAYKLVDVPELGYTTKDKPFPRGELRIKTRRMIPGYYKHPEATADLFDEEGFLKTGDVVEQRDADTFIWLDRVKNIIKLSQGEYVSVSRLEEIYVGNSKLIHQMYIYGNSLRAYLVAVVVPHIENGACADAGKLRAALRTELDDVARRKALQGYEIPREFIVEMRPFSKDNHLLTDSAKPARGQLKKRYQAELEGLYTALEERLRERLRAMKEGKDASVQDRIKQALEVTLGLAEEDMADVASRSFAQLGGDSLAAIQFARYVGELCGVNLPVSFVLDHSHSLQAIADRVHELVSGDASAGITFESIHGSDGVNIKAADLKLDRFLSEADTAAAAAAAPASELPARPTHVLLTGANGFLGRFLLLDLLQRGSDKNGGRVVAIVRGSSDEKAAERLRAGFDSGDATLLQRYDTLSKHLTVYAGDLAKPQLGLSQGVYESLCAELDTIVHNGALVNHAYSYEQLFEPNVLGSVEVMRMALAKRRKALTFISSVGVVGGLDHPQPVTEAEDGPTLCDVHPGDGGYAIGYGCSKWAVEVLLKELHQRWGVPVKVFRCGMILSHTSYLGQINPTDFFTRLLCGIAYTGIAPQSFYTLPHGPEEHFDGMPIDFVSGVISATTAAERSGFDTYHVVNPHWSDGVSLDRIVDWAESAGYPVNRIAPYEQWYAQFKAALEALDHTRQQQSPLPIIYQWERPASGTSGTKYDATQLRKRAAAYTQWKDVPHLDEAFIHQNMRHLTTLRLITPPGKA

SEQ ID NO: 84 - DNA, 4717 bp, Artificial Sequence
  Nucleotide sequence of DNA fragment containing ACAR gene of Coccomyxa subellipsoidea (codon-optimized) and entD gene of Escherichia coli
ccaagcttgcatgccagatcgtttagatccgaaggaaaacgtcgaaaagcaatttgcttttcgacgccccaccccgcgcgttttagcgtgtcagtagacgcgtagggtaagtggggtagcggcttgttagatatcttgaaatcggctttcaacagcattgatttcgatgtatttagctggccgtttgagacgcgatgtccacagggtagctggtagtttgaaaatcaacgccgttgcccttaggattcagtaactggcacattttgtaatgcgctagatctgtgtgcccagtcttccaggctgcttatcacagtgaaagcaaaaccaattcgtggctgcgaaagtcgtagccaccacgaagtccaggaggacatacaatgaccgaaaatggtggtctgccgcaggttaatggtggtggtccgcagtattgggaaatgagcaatggtcagaatcagaccaataacgtgattcagaaacgtctggcacgtgcgcgtgaagttattaaacaggatccgcagctgcaggcagcaaaatttgatcgtaaaagcctgcagcgtattaccgatgcaggtaataccagcattgaaattattgcagccatgtttaaagaatacgcaagccgtgacctgtttggtgcatgtacaccgggtgaaagcacctttcataccgttacctatggtgcagtttgggaacgtattcaggcactggttgcaggttggaccgcactgggttttgttgctccgggtgattttgttggtattagcggttttgcaagcgttgattgggttgttagcgatctggcaaccctgcatgccggtggtgttatggttccgctgccgaccaatattctggccgaagatgttcgtgcaattattgatgaagccgaagttcgttgtctgatggttagcgcagaagaactggcagcaattgcaccggttattggtggttgtgccagcgttaaagcagttattgttatggatagcagcaccgatgccgttaccagcagcggtgcatatgccgaaatgcaggccaatctgcctgccggtgcaaaactgaccaccatcgatgaagttctggcagcaggtcgtgcaaccggtaaacagcctgccctggttattccgggtcgtgatggtcgtccggcagatccgctggttaatctgatgtataccagcggtagcagcggtcgtccgaaaggtgcagaatatccggaacatctgatttttgattttctgaaaaatagcatgccgaccgatgcaccggaactgccgacgattattatgggttttctgccgctgaatcatctgatgggtcgttttaccctgctgaaatgtctgctgaccggtggccagaattggtttgttcgtagcaccgatatgagcaccttttttgatgatctggcgaccattcgtccgaccgaagcaatgtttccgcctcgtattatgaatatgctgcatgatcgttttgtggaacagctggatcgtctgcctccggcaccgagcgaagcagaacgtgcacagcagcgtcaggatctgattaaacgttttcgtgaagttgatctgggtggtcgtctgtttacaggtagctttggtagcgcaccggcaagtccggatgttattcagtggctggaagaagtgctgggttttccgcctgttaatggttatggtagtaccgaaggtggtatgattatgctggacaacaaaattcagcacagctatgttccagcctataaactggttgatgtgccggaactgggttataccaccaaagataaaccgtttccgcgtggtgaactgcgtattaaaacccgtcgtatgattccgggttattacaaacatcctgaagcaaccgcagacctgttcgatgaagaaggtttcctgaaaaccggtgatgttgttgaacagcgtgatgcagatacctttatttggctggatcgcgtgaaaaacattatcaaactgagccagggtgaatatgttagcgttagccgtctggaagaaatttatgtgggtaacagcaaactgattcaccagatgtatatctatggtaatagcctgcgtgcatatctggttgccgttgttgttccgcatattgaaaatggcgcatgtgcagatgccggtaaactgcgtgcagcactgcgtaccgaactggatgatgttgcacgtcgtaaagcactgcagggttatgaaattcctcgtgaatttattgttgagatgcgtccgtttagcaaagataatcatctgctgacagatagcgcaaaaccggcacgtggtcagctgaaaaaacgttatcaggcagaactggaaggtctgtatacggcactggaagaacgtctgcgtgaacggctgcgtgcaatgaaagaaggtaaagacgcaagcgttcaggatcgtatcaaacaggccctggaagttaccctgggtctggcggaagaggatatggcagatgttgcaagccgtagctttgcacagctgggtggtgatagcctggcagccattcagtttgcacgttatgttggcgaactgtgtggtgttaatctgccggttagctttgttctggatcatagccatagtctgcaggcaattgcagatcgtgtgcatgaactggttagcggtgatgcctcagcaggcattacctttgaaagcattcatggtagtgatggcgttaacattaaagcagcagatctgaaactggatcgttttctgagcgaagccgataccgcagcagcagccgctgcagcaccggcatcagaactgcctgcacgtccgacccatgttctgctgactggcgcaaatggttttctgggtcgctttctgctgctggatctgctgcagcgtggtagcgataaaaatggcggtcgtgttgttgcaattgttcgtggtagcagtgatgaaaaagcagccgaacgcctgcgtgcgggttttgatagtggtgatgccaccctgctgcaacgttatgataccctgagcaaacatctgaccgtttatgccggtgatctggccaaaccgcagctgggtctgagtcagggtgtttatgaaagcctgtgtgcagagctggataccattgttcataatggtgcactggtgaaccatgcctatagctatgagcagctgtttgaaccgaatgttctgggtagcgttgaagttatgcgtatggcactggcaaaacgccgtaaagccctgacctttattagcagcgttggtgttgtgggtggcctggatcatccgcagccggttaccgaagcggaagatggtccgaccctgtgtgatgttcatcctggtgatggtggttatgcaattggttatggctgtagcaaatgggcagttgaagtgctgctgaaagaactgcatcagcgttggggtgttccggttaaagtttttcgttgcggtatgattctgtcccataccagctatctgggtcagattaatccgacagattttttcacccgtctgctgtgtggtattgcatatacaggtattgcaccgcagagcttttataccctgccgcatggtccggaagaacattttgatggtatgccgattgattttgtgagcggtgttattagcgcaaccacagccgcagaacgtagcggctttgatacctatcatgttgttaatccgcattggagtgatggtgtgagcctggatcgtattgtagattgggcagaaagtgcaggttatccggttaatcgtatcgcaccgtacgaacagtggtatgcacagtttaaagcagccctggaagcactggatcatacccgtcagcagcagtcaccgctgccgattatctatcagtgggaacgtccggcaagcggtacaagcggcaccaaatatgatgcaacacagctgcgtaaacgtgcagcagcctatacccagtggaaagatgtgccgcatctggatgaagcatttattcatcagaatatgcgtcatctgaccaccctgcgtctgattacccctccgggtaaagcataaaggaggacatacaatggtcgatatgaaaactacgcatacctccctcccctttgccggacatacgctgcattttgttgagttcgatccggcgaatttttgtgagcaggatttactctggctgccgcactacgcacaactgcaacacgctggacgtaaacgtaaaacagagcatttagccggacggatcgctgctgtttatgctttgcgggaatatggctataaatgtgtgcccgcaatcggcgagctacgccaacctgtctggcctgcggaggtatacggcagtattagccactgtgggactacggcattagccgtggtatctcgtcaaccgattggcattgatatagaagaaattttttctgtacaaaccgcaagagaattgacagacaacattattacaccagcggaacacgagcgactcgcagactgcggtttagccttttctctggcgctgacactggcattttccgccaaagagagcgcatttaaggcaagtgagatccaaactgatgcaggttttctggactatcagataattagctggaataaacagcaggtcatcattcatcgtgagaatgagatgtttgctgtgcactggcagataaaagaaaagatagtcataacgctgtgccaacacgattaattgacaacatctggtacgattcgcccgcagccatcactgaccacgggcgaaagtgtaaagcaggtgccttaccatcctgacctgacaaccggatatgcgggatccccgggtaccg

SEQ ID NO: 85 - DNA, 3582 bp, Coccomyxa subellipsoidea
atgaccgaaaatggtggtctgccgcaggttaatggtggtggtccgcagtattgggaaatgagcaatggtcagaatcagaccaataacgtgattcagaaacgtctggcacgtgcgcgtgaagttattaaacaggatccgcagctgcaggcagcaaaatttgatcgtaaaagcctgcagcgtattaccgatgcaggtaataccagcattgaaattattgcagccatgtttaaagaatacgcaagccgtgacctgtttggtgcatgtacaccgggtgaaagcacctttcataccgttacctatggtgcagtttgggaacgtattcaggcactggttgcaggttggaccgcactgggttttgttgctccgggtgattttgttggtattagcggttttgcaagcgttgattgggttgttagcgatctggcaaccctgcatgccggtggtgttatggttccgctgccgaccaatattctggccgaagatgttcgtgcaattattgatgaagccgaagttcgttgtctgatggttagcgcagaagaactggcagcaattgcaccggttattggtggttgtgccagcgttaaagcagttattgttatggatagcagcaccgatgccgttaccagcagcggtgcatatgccgaaatgcaggccaatctgcctgccggtgcaaaactgaccaccatcgatgaagttctggcagcaggtcgtgcaaccggtaaacagcctgccctggttattccgggtcgtgatggtcgtccggcagatccgctggttaatctgatgtataccagcggtagcagcggtcgtccgaaaggtgcagaatatccggaacatctgatttttgattttctgaaaaatagcatgccgaccgatgcaccggaactgccgacgattattatgggttttctgccgctgaatcatctgatgggtcgttttaccctgctgaaatgtctgctgaccggtggccagaattggtttgttcgtagcaccgatatgagcaccttttttgatgatctggcgaccattcgtccgaccgaagcaatgtttccgcctcgtattatgaatatgctgcatgatcgttttgtggaacagctggatcgtctgcctccggcaccgagcgaagcagaacgtgcacagcagcgtcaggatctgattaaacgttttcgtgaagttgatctgggtggtcgtctgtttacaggtagctttggtagcgcaccggcaagtccggatgttattcagtggctggaagaagtgctgggttttccgcctgttaatggttatggtagtaccgaaggtggtatgattatgctggacaacaaaattcagcacagctatgttccagcctataaactggttgatgtgccggaactgggttataccaccaaagataaaccgtttccgcgtggtgaactgcgtattaaaacccgtcgtatgattccgggttattacaaacatcctgaagcaaccgcagacctgttcgatgaagaaggtttcctgaaaaccggtgatgttgttgaacagcgtgatgcagatacctttatttggctggatcgcgtgaaaaacattatcaaactgagccagggtgaatatgttagcgttagccgtctggaagaaatttatgtgggtaacagcaaactgattcaccagatgtatatctatggtaatagcctgcgtgcatatctggttgccgttgttgttccgcatattgaaaatggcgcatgtgcagatgccggtaaactgcgtgcagcactgcgtaccgaactggatgatgttgcacgtcgtaaagcactgcagggttatgaaattcctcgtgaatttattgttgagatgcgtccgtttagcaaagataatcatctgctgacagatagcgcaaaaccggcacgtggtcagctgaaaaaacgttatcaggcagaactggaaggtctgtatacggcactggaagaacgtctgcgtgaacggctgcgtgcaatgaaagaaggtaaagacgcaagcgttcaggatcgtatcaaacaggccctggaagttaccctgggtctggcggaagaggatatggcagatgttgcaagccgtagctttgcacagctgggtggtgatagcctggcagccattcagtttgcacgttatgttggcgaactgtgtggtgttaatctgccggttagctttgttctggatcatagccatagtctgcaggcaattgcagatcgtgtgcatgaactggttagcggtgatgcctcagcaggcattacctttgaaagcattcatggtagtgatggcgttaacattaaagcagcagatctgaaactggatcgttttctgagcgaagccgataccgcagcagcagccgctgcagcaccggcatcagaactgcctgcacgtccgacccatgttctgctgactggcgcaaatggttttctgggtcgctttctgctgctggatctgctgcagcgtggtagcgataaaaatggcggtcgtgttgttgcaattgttcgtggtagcagtgatgaaaaagcagccgaacgcctgcgtgcgggttttgatagtggtgatgccaccctgctgcaacgttatgataccctgagcaaacatctgaccgtttatgccggtgatctggccaaaccgcagctgggtctgagtcagggtgtttatgaaagcctgtgtgcagagctggataccattgttcataatggtgcactggtgaaccatgcctatagctatgagcagctgtttgaaccgaatgttctgggtagcgttgaagttatgcgtatggcactggcaaaacgccgtaaagccctgacctttattagcagcgttggtgttgtgggtggcctggatcatccgcagccggttaccgaagcggaagatggtccgaccctgtgtgatgttcatcctggtgatggtggttatgcaattggttatggctgtagcaaatgggcagttgaagtgctgctgaaagaactgcatcagcgttggggtgttccggttaaagtttttcgttgcggtatgattctgtcccataccagctatctgggtcagattaatccgacagattttttcacccgtctgctgtgtggtattgcatatacaggtattgcaccgcagagcttttataccctgccgcatggtccggaagaacattttgatggtatgccgattgattttgtgagcggtgttattagcgcaaccacagccgcagaacgtagcggctttgatacctatcatgttgttaatccgcattggagtgatggtgtgagcctggatcgtattgtagattgggcagaaagtgcaggttatccggttaatcgtatcgcaccgtacgaacagtggtatgcacagtttaaagcagccctggaagcactggatcatacccgtcagcagcagtcaccgctgccgattatctatcagtgggaacgtccggcaagcggtacaagcggcaccaaatatgatgcaacacagctgcgtaaacgtgcagcagcctatacccagtggaaagatgtgccgcatctggatgaagcatttattcatcagaatatgcgtcatctgaccaccctgcgtctgattacccctccgggtaaagcataa